European Patent Application EP 4 279 584 A2, published November 22, 2023. Title: COMPOSITIONS AND METHODS FOR TREATING CANCER WITH ANTI-CD22 IMMUNOTHERAPY. Applicant: Lentigen Technology, Inc. Application EP, filed July 25, 2023. The sequence listing filed with the application follows.

SEQUENCE LISTING (206 sequences)

SEQ ID NO: 1 - DNA, 732 bp, synthetic construct
  misc_feature 1..732: note = Description of Artificial Sequence: Synthetic polynucleotide
  source 1..732: mol_type = other DNA
caagtacaactccagcaaagcgggcctggtctggtgaagccgtcacagacgctttcacttacgtgtgcgatctccggtgactccgtgagttctaatagcgcggcttggaactggattaggcagtctccatcccgaggattggaatggctcggcaggacttattatagaagtaagtggtacaacgattatgcagtctctgtgaaatctcgcatcaccattaacccagacacgtctaagaatcagttcagtcttcaactcaactctgtaacccccgaagatacagcggtctactactgtgctcaggaggtgcaaccccacgatgcttttgatatctggggccagggtaccatggttacggtgtcttctgggggaggggggtccggtgggggaggatcagggggtgggggcagcgacatacaaatgacgcaatccccgtcttctgtttctgcgtctgtcggagataaagtaacaataacctgtcgagcgtcacaggacgttagtggctggcttgcgtggtatcagcaaaaaccggggctcgccccgcaattgcttatatttggagcgagtactcttcagggcgaggtacctagcagattttctgggtccggctcaggtacggacttcaccctgaccatatctagcttgcagcctgaagatttcgccacctactattgtcaacaggcgaagaactttccatatacgttcgggcagggtacgaaattggagataaaa

SEQ ID NO: 2 - protein, 245 aa, synthetic construct
  REGION 1..245: note = Description of Artificial Sequence: Synthetic polypeptide
QVQLQQSGPGLVKPSQTLSLTCAISGDSVSSNSAAWNWIRQSPSRGLEWLGRTYYRSKWYNDYAVSVKSRITINPDTSKNQFSLQLNSVTPEDTAVYYCAQEVQPHDAFDIWGQGTMVTVSSGGGGSGGGGSGGGGSDIQMTQSPSSVSASVGDKVTITCRASQDVSGWLAWYQQKPGLAPQLLIFGASTLQGEVPSRFSGSGSGTDFTLTISSLQPEDFATYYCQQAKNFPYTFGQGTKLEIKR

SEQ ID NO: 3 - DNA, 1476 bp, synthetic construct
  misc_feature 1..1476: note = Description of Artificial Sequence: Synthetic polynucleotide
  source 1..1476: mol_type = other DNA
atgcttctcctggtgacaagccttctgctctgtgagttaccacacccagcattcctcctgatcccacaagtacaactccagcaaagcgggcctggtctggtgaagccgtcacagacgctttcacttacgtgtgcgatctccggtgactccgtgagttctaatagcgcggcttggaactggattaggcagtctccatcccgaggattggaatggctcggcaggacttattatagaagtaagtggtacaacgattatgcagtctctgtgaaatctcgcatcaccattaacccagacacgtctaagaatcagttcagtcttcaactcaactctgtaacccccgaagatacagcggtctactactgtgctcaggaggtgcaaccccacgatgcttttgatatctggggccagggtaccatggttacggtgtcttctgggggaggggggtccggtgggggaggatcagggggtgggggcagcgacatacaaatgacgcaatccccgtcttctgtttctgcgtctgtcggagataaagtaacaataacctgtcgagcgtcacaggacgttagtggctggcttgcgtggtatcagcaaaaaccggggctcgccccgcaattgcttatatttggagcgagtactcttcagggcgaggtacctagcagattttctgggtccggctcaggtacggacttcaccctgaccatatctagcttgcagcctgaagatttcgccacctactattgtcaacaggcgaagaactttccatatacgttcgggcagggtacgaaattggagataaaagcggccgcaactaccacccctgcccctcggccgccgactccggccccaaccatcgcaagccaacccctctccttgcgccccgaagcttgccgcccggccgcgggtggagccgtgcatacccgggggctggactttgcctgcgatatctacatttgggccccgctggccggcacttgcggcgtgctcctgctgtcgctggtcatcaccctttactgcaagaggggccggaagaagctgctttacatcttcaagcagccgttcatgcggcccgtgcagacgactcaggaagaggacggatgctcgtgcagattccctgaggaggaagaggggggatgcgaactgcgcgtcaagttctcacggtccgccgacgcccccgcatatcaacagggccagaatcagctctacaacgagctgaacctgggaaggagagaggagtacgacgtgctggacaagcgacgcggacgcgacccggagatgggggggaaaccacggcggaaaaaccctcaggaaggactgtacaacgaactccagaaagacaagatggcggaagcctactcagaaatcgggatgaagggagagcggaggaggggaaagggtcacgacgggctgtaccagggactgagcaccgccactaaggatacctacgatgccttgcatatgcaagcactcccaccccgg

SEQ ID NO: 4 - protein, 492 aa, synthetic construct
  REGION 1..492: note = Description of Artificial Sequence: Synthetic polypeptide
MLLLVTSLLLCELPHPAFLLIPQVQLQQSGPGLVKPSQTLSLTCAISGDSVSSNSAAWNWIRQSPSRGLEWLGRTYYRSKWYNDYAVSVKSRITINPDTSKNQFSLQLNSVTPEDTAVYYCAQEVQPHDAFDIWGQGTMVTVSSGGGGSGGGGSGGGGSDIQMTQSPSSVSASVGDKVTITCRASQDVSGWLAWYQQKPGLAPQLLIFGASTLQGEVPSRFSGSGSGTDFTLTISSLQPEDFATYYCQQAKNFPYTFGQGTKLEIKAAATTTPAPRPPTPAPTIASQPLSLRPEACRPAAGGAVHTRGLDFACDIYIWAPLAGTCGVLLLSLVITLYCKRGRKKLLYIFKQPFMRPVQTTQEEDGCSCRFPEEEEGGCELRVKFSRSADAPAYQQGQNQLYNELNLGRREEYDVLDKRRGRDPEMGGKPRRKNPQEGLYNELQKDKMAEAYSEIGMKGERRRGKGHDGLYQGLSTATKDTYDALHMQALPPR

SEQ ID NO: 5 - protein, 6 aa, synthetic construct
  REGION 1..6: note = Description of Artificial Sequence: Synthetic peptide
QDVSGW

SEQ ID NO: 6 - skipped

SEQ ID NO: 7 - protein, 9 aa, synthetic construct
  REGION 1..9: note = Description of Artificial Sequence: Synthetic peptide
QQAKNFPYT

SEQ ID NO: 8 - protein, 10 aa, synthetic construct
  REGION 1..10: note = Description of Artificial Sequence: Synthetic peptide
GDSVSSNSAA

SEQ ID NO: 9 - protein, 9 aa, synthetic construct
  REGION 1..9: note = Description of Artificial Sequence: Synthetic peptide
TYYRSKWYN

SEQ ID NO: 10 - protein, 12 aa, synthetic construct
  REGION 1..12: note = Description of Artificial Sequence: Synthetic peptide
AQEVQPHDAFDI

SEQ ID NO: 11 - DNA, 732 bp, synthetic construct
  misc_feature 1..732: note = Description of Artificial Sequence: Synthetic polynucleotide
  source 1..732: mol_type = other DNA
caagtacagctgcaacaatctggccctgggcttgtgaaaccctctcagactttgtccttgacgtgcgcgataagtggcgattcagttagttctaacagcgccgcttggaactggattagacagagccccagtcggggactcgaatggcttggccggacttattatcgcagtaaatggtataatgattatgctgtgagtgtgaaaagtaggatcacaatcaaccccgatacgagcaagaatcaattctcattgcaactgaacagcgtcactcccgaggatacagctgtatattattgtgcaagagaaggtgggtggtatggcgagatggatgtatgggggaaaggaactacggtaactgtgtccagtggcggaggcggttcaggtggtggaggctctggaggaggagggtccgaaatcgtgcttacccagtctccggctactctgagcgttagtccgggtgaaagggcctcactctcttgtcgagcttcacagtcagtctcttcctacttggcttggtatcagcagaagccaggtcaggcgccccgcttgctcatttacgacgcaagcacacgagcgacaggcattccagacagattttctggttctggttctggcacggactttactcttactataaactcacttgaggcagaggatgctgcgacttactattgtcaccaatcaagctctctgccttacacctttgggcaaggcaccaaactcgaaatcaag

SEQ ID NO: 12 - protein, 245 aa, synthetic construct
  REGION 1..245: note = Description of Artificial Sequence: Synthetic polypeptide
QVQLQQSGPGLVKPSQTLSLTCAISGDSVSSNSAAWNWIRQSPSRGLEWLGRTYYRSKWYNDYAVSVKSRITINPDTSKNQFSLQLNSVTPEDTAVYYCAREGGWYGEMDVWGKGTTVTVSSGGGGSGGGGSGGGGSEIVLTQSPATLSVSPGERASLSCRASQSVSSYLAWYQQKPGQAPRLLIYDASTRATGIPDRFSGSGSGTDFTLTINSLEAEDAATYYCHQSSSLPYTFGQGTKLEIKR

SEQ ID NO: 13 - DNA, 1491 bp, synthetic construct
  misc_feature 1..1491: note = Description of Artificial Sequence: Synthetic polynucleotide
  source 1..1491: mol_type = other DNA
atgctgctgttggtgacatcacttctgctctgtgaactcccccatccagcctttctgcttataccgcaagtacagctgcaacaatctggccctgggcttgtgaaaccctctcagactttgtccttgacgtgcgcgataagtggcgattcagttagttctaacagcgccgcttggaactggattagacagagccccagtcggggactcgaatggcttggccggacttattatcgcagtaaatggtataatgattatgctgtgagtgtgaaaagtaggatcacaatcaaccccgatacgagcaagaatcaattctcattgcaactgaacagcgtcactcccgaggatacagctgtatattattgtgcaagagaaggtgggtggtatggcgagatggatgtatgggggaaaggaactacggtaactgtgtccagtggcggaggcggttcaggtggtggaggctctggaggaggagggtccgaaatcgtgcttacccagtctccggctactctgagcgttagtccgggtgaaagggcctcactctcttgtcgagcttcacagtcagtctcttcctacttggcttggtatcagcagaagccaggtcaggcgccccgcttgctcatttacgacgcaagcacacgagcgacaggcattccagacagattttctggttctggttctggcacggactttactcttactataaactcacttgaggcagaggatgctgcgacttactattgtcaccaatcaagctctctgccttacacctttgggcaaggcaccaaactcgaaatcaaggttacggtatcatctgcggccgcaactaccacccctgcccctcggccgccgactccggccccaaccatcgcaagccaacccctctccttgcgccccgaagcttgccgcccggccgcgggtggagccgtgcatacccgggggctggactttgcctgcgatatctacatttgggccccgctggccggcacttgcggcgtgctcctgctgtcgctggtcatcaccctttactgcaagaggggccggaagaagctgctttacatcttcaagcagccgttcatgcggcccgtgcagacgactcaggaagaggacggatgctcgtgcagattccctgaggaggaagaggggggatgcgaactgcgcgtcaagttctcacggtccgccgacgcccccgcatatcaacagggccagaatcagctctacaacgagctgaacctgggaaggagagaggagtacgacgtgctggacaagcgacgcggacgcgacccggagatgggggggaaaccacggcggaaaaaccctcaggaaggactgtacaacgaactccagaaagacaagatggcggaagcctactcagaaatcgggatgaagggagagcggaggaggggaaagggtcacgacgggctgtaccagggactgagcaccgccactaaggatacctacgatgccttgcatatgcaagcactcccaccccgg

SEQ ID NO: 14 - protein, 497 aa, synthetic construct
  REGION 1..497: note = Description of Artificial Sequence: Synthetic polypeptide
MLLLVTSLLLCELPHPAFLLIPQVQLQQSGPGLVKPSQTLSLTCAISGDSVSSNSAAWNWIRQSPSRGLEWLGRTYYRSKWYNDYAVSVKSRITINPDTSKNQFSLQLNSVTPEDTAVYYCAREGGWYGEMDVWGKGTTVTVSSGGGGSGGGGSGGGGSEIVLTQSPATLSVSPGERASLSCRASQSVSSYLAWYQQKPGQAPRLLIYDASTRATGIPDRFSGSGSGTDFTLTINSLEAEDAATYYCHQSSSLPYTFGQGTKLEIKVTVSSAAATTTPAPRPPTPAPTIASQPLSLRPEACRPAAGGAVHTRGLDFACDIYIWAPLAGTCGVLLLSLVITLYCKRGRKKLLYIFKQPFMRPVQTTQEEDGCSCRFPEEEEGGCELRVKFSRSADAPAYQQGQNQLYNELNLGRREEYDVLDKRRGRDPEMGGKPRRKNPQEGLYNELQKDKMAEAYSEIGMKGERRRGKGHDGLYQGLSTATKDTYDALHMQALPPR

SEQ ID NO: 15 - protein, 6 aa, synthetic construct
  REGION 1..6: note = Description of Artificial Sequence: Synthetic peptide
QSVSSY

SEQ ID NO: 16 - skipped

SEQ ID NO: 17 - protein, 9 aa, synthetic construct
  REGION 1..9: note = Description of Artificial Sequence: Synthetic peptide
HQSSSLPYT

SEQ ID NO: 18 - protein, 10 aa, synthetic construct
  REGION 1..10: note = Description of Artificial Sequence: Synthetic peptide
GDSVSSNSAA

SEQ ID NO: 19 - protein, 9 aa, synthetic construct
  REGION 1..9: note = Description of Artificial Sequence: Synthetic peptide
TYYRSKWYN

SEQ ID NO: 20 - protein, 12 aa, synthetic construct
  REGION 1..12: note = Description of Artificial Sequence: Synthetic peptide
AREGGWYGEMDV

SEQ ID NO: 21 - DNA, 744 bp, synthetic construct
  misc_feature 1..744: note = Description of Artificial Sequence: Synthetic polynucleotide
  source 1..744: mol_type = other DNA
caagtacagctccaacagagtggacctggtctcgttaagccgtcccaaacactgtctttgacgtgcgctattagtggcgacagcgtatcatccaattctgctgcttggaactggattagacagtcaccgtccagaggcttggaatggctgggcaggacgtactaccgctcaaaatggtataacgattacgcggttagtgtcaaatccaggattaccattaaccctgacacaagtaagaatcagttttctcttcagctgaattccctgactcctgaggatacggccgtttactactgtgcccgagaacaccagaatgaggcggcttttgatatttgggggcaaggaacaatggtcacagttagcagtggggggggtggctccgggggaggtggttccggcggcggtggttctcaatccgtcctgacacaacctccctcagcgagcgggactcccggtcaaagggtgaccatctcttgttctgggggaggtagtaacatcgggacaaatactgcgtcctggtatcagcaactccctgggaccgctcccaagttgttgatatatcgcaatacgcaacgacctagtgggatacctgatagattcagcggaagcaaaagtggtacgagtgcgtctttggcaatatctggcctccagtccgaggacgaagcggattactattgtgcggcctgggatgactcactgaatggttatgtgttcggtgcaggtactcaactcaccgtacttggt

SEQ ID NO: 22 - protein, 248 aa, synthetic construct
  REGION 1..248: note = Description of Artificial Sequence: Synthetic polypeptide
QVQLQQSGPGLVKPSQTLSLTCAISGDSVSSNSAAWNWIRQSPSRGLEWLGRTYYRSKWYNDYAVSVKSRITINPDTSKNQFSLQLNSLTPEDTAVYYCAREHQNEAAFDIWGQGTMVTVSSGGGGSGGGGSGGGGSQSVLTQPPSASGTPGQRVTISCSGGGSNIGTNTASWYQQLPGTAPKLLIYRNTQRPSGIPDRFSGSKSGTSASLAISGLQSEDEADYYCAAWDDSLNGYVFGAGTQLTVLG

SEQ ID NO: 23 - DNA, 1488 bp, synthetic construct
  misc_feature 1..1488: note = Description of Artificial Sequence: Synthetic polynucleotide
  source 1..1488: mol_type = other DNA
atgcttctcctggtgacaagccttctgctctgtgagttaccacacccagcattcctcctgatcccacaagtacagctccaacagagtggacctggtctcgttaagccgtcccaaacactgtctttgacgtgcgctattagtggcgacagcgtatcatccaattctgctgcttggaactggattagacagtcaccgtccagaggcttggaatggctgggcaggacgtactaccgctcaaaatggtataacgattacgcggttagtgtcaaatccaggattaccattaaccctgacacaagtaagaatcagttttctcttcagctgaattccctgactcctgaggatacggccgtttactactgtgcccgagaacaccagaatgaggcggcttttgatatttgggggcaaggaacaatggtcacagttagcagtggggggggtggctccgggggaggtggttccggcggcggtggttctcaatccgtcctgacacaacctccctcagcgagcgggactcccggtcaaagggtgaccatctcttgttctgggggaggtagtaacatcgggacaaatactgcgtcctggtatcagcaactccctgggaccgctcccaagttgttgatatatcgcaatacgcaacgacctagtgggatacctgatagattcagcggaagcaaaagtggtacgagtgcgtctttggcaatatctggcctccagtccgaggacgaagcggattactattgtgcggcctgggatgactcactgaatggttatgtgttcggtgcaggtactcaactcaccgtacttggtgcggccgcaactaccacccctgcccctcggccgccgactccggccccaaccatcgcaagccaacccctctccttgcgccccgaagcttgccgcccggccgcgggtggagccgtgcatacccgggggctggactttgcctgcgatatctacatttgggccccgctggccggcacttgcggcgtgctcctgctgtcgctggtcatcaccctttactgcaagaggggccggaagaagctgctttacatcttcaagcagccgttcatgcggcccgtgcagacgactcaggaagaggacggatgctcgtgcagattccctgaggaggaagaggggggatgcgaactgcgcgtcaagttctcacggtccgccgacgcccccgcatatcaacagggccagaatcagctctacaacgagctgaacctgggaaggagagaggagtacgacgtgctggacaagcgacgcggacgcgacccggagatgggggggaaaccacggcggaaaaaccctcaggaaggactgtacaacgaactccagaaagacaagatggcggaagcctactcagaaatcgggatgaagggagagcggaggaggggaaagggtcacgacgggctgtaccagggactgagcaccgccactaaggatacctacgatgccttgcatatgcaagcactcccaccccgg

SEQ ID NO: 24 - protein, 496 aa, synthetic construct
  REGION 1..496: note = Description of Artificial Sequence: Synthetic polypeptide
MLLLVTSLLLCELPHPAFLLIPQVQLQQSGPGLVKPSQTLSLTCAISGDSVSSNSAAWNWIRQSPSRGLEWLGRTYYRSKWYNDYAVSVKSRITINPDTSKNQFSLQLNSLTPEDTAVYYCAREHQNEAAFDIWGQGTMVTVSSGGGGSGGGGSGGGGSQSVLTQPPSASGTPGQRVTISCSGGGSNIGTNTASWYQQLPGTAPKLLIYRNTQRPSGIPDRFSGSKSGTSASLAISGLQSEDEADYYCAAWDDSLNGYVFGAGTQLTVLGAAATTTPAPRPPTPAPTIASQPLSLRPEACRPAAGGAVHTRGLDFACDIYIWAPLAGTCGVLLLSLVITLYCKRGRKKLLYIFKQPFMRPVQTTQEEDGCSCRFPEEEEGGCELRVKFSRSADAPAYQQGQNQLYNELNLGRREEYDVLDKRRGRDPEMGGKPRRKNPQEGLYNELQKDKMAEAYSEIGMKGERRRGKGHDGLYQGLSTATKDTYDALHMQALPPR

SEQ ID NO: 25 - protein, 8 aa, synthetic construct
  REGION 1..8: note = Description of Artificial Sequence: Synthetic peptide
GSNIGTNT

SEQ ID NO: 26 - skipped

SEQ ID NO: 27 - protein, 11 aa, synthetic construct
  REGION 1..11: note = Description of Artificial Sequence: Synthetic peptide
AAWDDSLNGYV

SEQ ID NO: 28 - protein, 10 aa, synthetic construct
  REGION 1..10: note = Description of Artificial Sequence: Synthetic peptide
GDSVSSNSAA

SEQ ID NO: 29 - protein, 9 aa, synthetic construct
  REGION 1..9: note = Description of Artificial Sequence: Synthetic peptide
TYYRSKWYN

SEQ ID NO: 30 - protein, 12 aa, synthetic construct
  REGION 1..12: note = Description of Artificial Sequence: Synthetic peptide
AREHQNEAAFDI

SEQ ID NO: 31 - DNA, 729 bp, synthetic construct
  misc_feature 1..729: note = Description of Artificial Sequence: Synthetic polynucleotide
  source 1..729: mol_type = other DNA
caagtccagttgcaacagtccgggccaggtctggttaagccatcccaaactctgagtttgacgtgcgctattagcggagattccgtgtccagcaattctgcaacctggaattggatccggcagagtccgagtggcggtttggaatggctcggacgcacttactacaggagcaaatggtacgatgattatgctgtttctgtgcgctctcgaatcaccatgaatcctgatacttctaagaaccaattttctttgcagttgaactccgtcacgcctgaagatactgcggtctactattgcgcacgcgaaggcgtagccggcgattttgattactgggggcaaggaacattggtcacggtctcctctggtggaggaggatcaggaggcgggggttcaggtggaggtgggagcgatattcaacttacgcagtctccgagcagtctttctgcttccgtgggagaccgagtgacgattacttgtagggcatctcagtcaataagttcctatcttaactggtatcagcagaagcctggaaaggctccaaaacttcttatttatgccgcatcctcattgcaatccggcgtgccttcccgattttccggatctggctcaggcactgactttaccttgactattagttcccttcaaccagaagattttgctacctattactgccaacaatcatacagtaccccatatacattcggccaaggcacgaaattggagattaaa

SEQ ID NO: 32 - protein, 244 aa, synthetic construct
  REGION 1..244: note = Description of Artificial Sequence: Synthetic polypeptide
QVQLQQSGPGLVKPSQTLSLTCAISGDSVSSNSATWNWIRQSPSGGLEWLGRTYYRSKWYDDYAVSVRSRITMNPDTSKNQFSLQLNSVTPEDTAVYYCAREGVAGDFDYWGQGTLVTVSSGGGGSGGGGSGGGGSDIQLTQSPSSLSASVGDRVTITCRASQSISSYLNWYQQKPGKAPKLLIYAASSLQSGVPSRFSGSGSGTDFTLTISSLQPEDFATYYCQQSYSTPYTFGQGTKLEIKR

SEQ ID NO: 33 - DNA, 1473 bp, synthetic construct
  misc_feature 1..1473: note = Description of Artificial Sequence: Synthetic polynucleotide
  source 1..1473: mol_type = other DNA
atgcttctcctggtgacaagccttctgctctgtgagttaccacacccagcattcctcctgatcccacaagtccagttgcaacagtccgggccaggtctggttaagccatcccaaactctgagtttgacgtgcgctattagcggagattccgtgtccagcaattctgcaacctggaattggatccggcagagtccgagtggcggtttggaatggctcggacgcacttactacaggagcaaatggtacgatgattatgctgtttctgtgcgctctcgaatcaccatgaatcctgatacttctaagaaccaattttctttgcagttgaactccgtcacgcctgaagatactgcggtctactattgcgcacgcgaaggcgtagccggcgattttgattactgggggcaaggaacattggtcacggtctcctctggtggaggaggatcaggaggcgggggttcaggtggaggtgggagcgatattcaacttacgcagtctccgagcagtctttctgcttccgtgggagaccgagtgacgattacttgtagggcatctcagtcaataagttcctatcttaactggtatcagcagaagcctggaaaggctccaaaacttcttatttatgccgcatcctcattgcaatccggcgtgccttcccgattttccggatctggctcaggcactgactttaccttgactattagttcccttcaaccagaagattttgctacctattactgccaacaatcatacagtaccccatatacattcggccaaggcacgaaattggagattaaagcggccgcaactaccacccctgcccctcggccgccgactccggccccaaccatcgcaagccaacccctctccttgcgccccgaagcttgccgcccggccgcgggtggagccgtgcatacccgggggctggactttgcctgcgatatctacatttgggccccgctggccggcacttgcggcgtgctcctgctgtcgctggtcatcaccctttactgcaagaggggccggaagaagctgctttacatcttcaagcagccgttcatgcggcccgtgcagacgactcaggaagaggacggatgctcgtgcagattccctgaggaggaagaggggggatgcgaactgcgcgtcaagttctcacggtccgccgacgcccccgcatatcaacagggccagaatcagctctacaacgagctgaacctgggaaggagagaggagtacgacgtgctggacaagcgacgcggacgcgacccggagatgggggggaaaccacggcggaaaaaccctcaggaaggactgtacaacgaactccagaaagacaagatggcggaagcctactcagaaatcgggatgaagggagagcggaggaggggaaagggtcacgacgggctgtaccagggactgagcaccgccactaaggatacctacgatgccttgcatatgcaagcactcccaccccgg

SEQ ID NO: 34 - protein, 491 aa, synthetic construct
  REGION 1..491: note = Description of Artificial Sequence: Synthetic polypeptide
MLLLVTSLLLCELPHPAFLLIPQVQLQQSGPGLVKPSQTLSLTCAISGDSVSSNSATWNWIRQSPSGGLEWLGRTYYRSKWYDDYAVSVRSRITMNPDTSKNQFSLQLNSVTPEDTAVYYCAREGVAGDFDYWGQGTLVTVSSGGGGSGGGGSGGGGSDIQLTQSPSSLSASVGDRVTITCRASQSISSYLNWYQQKPGKAPKLLIYAASSLQSGVPSRFSGSGSGTDFTLTISSLQPEDFATYYCQQSYSTPYTFGQGTKLEIKAAATTTPAPRPPTPAPTIASQPLSLRPEACRPAAGGAVHTRGLDFACDIYIWAPLAGTCGVLLLSLVITLYCKRGRKKLLYIFKQPFMRPVQTTQEEDGCSCRFPEEEEGGCELRVKFSRSADAPAYQQGQNQLYNELNLGRREEYDVLDKRRGRDPEMGGKPRRKNPQEGLYNELQKDKMAEAYSEIGMKGERRRGKGHDGLYQGLSTATKDTYDALHMQALPPR

SEQ ID NO: 35 - protein, 6 aa, synthetic construct
  REGION 1..6: note = Description of Artificial Sequence: Synthetic peptide
QSISSY

SEQ ID NO: 36 - skipped

SEQ ID NO: 37 - protein, 9 aa, synthetic construct
  REGION 1..9: note = Description of Artificial Sequence: Synthetic peptide
QQSYSTPYT

SEQ ID NO: 38 - protein, 10 aa, synthetic construct
  REGION 1..10: note = Description of Artificial Sequence: Synthetic peptide
GDSVSSNSAT

SEQ ID NO: 39 - protein, 9 aa, synthetic construct
  REGION 1..9: note = Description of Artificial Sequence: Synthetic peptide
TYYRSKWYD

SEQ ID NO: 40 - protein, 11 aa, synthetic construct
  REGION 1..11: note = Description of Artificial Sequence: Synthetic peptide
AREGVAGDFDY

SEQ ID NO: 41 - DNA, 726 bp, synthetic construct
  misc_feature 1..726: note = Description of Artificial Sequence: Synthetic polynucleotide
  source 1..726: mol_type = other DNA
caagttcagttgcagcagagtggccctgggcttgttaaaccatcacagacgctctcactgacctgtgccatctctggagacagtgtaagttctaactcagccgcgtggaattggattagacaatcaccaagccggggacttgaatggcttggtcggacgtactatagatctaagtggtataatgactacgcagtgtcagtgaaatcacggataaccataaaccctgacaccagcaaaaaccaattttctcttcagcttaattccgtcacgccagaagatacggccgtttactactgtgcgagggaaggtgatgacgcattggacatctggggtcaggggaccatggtgactgtctcttccggcggggggggtagtggagggggtggctcaggtggtggcgggtcagatatacaaatgacacagagccctagtagtctgagtgcttcagtgggcgaccgcgtaactataacctgtagagcatcccaaagcatttcccacttccttaattggtaccagcagaagccgggcacagcgcccaaactcctgatcaccactgcgagcggacttggttcaggtgttcctagccggtttagtgggtcaggtagcggtacagatttcactctcacgataaactcccttcagcctgaggacctggcgacatattactgtcaacaatcctataccaccccactgacattcggagggggcacaaaactggagatcaaa

SEQ ID NO: 42 - protein, 243 aa, synthetic construct
  REGION 1..243: note = Description of Artificial Sequence: Synthetic polypeptide
QVQLQQSGPGLVKPSQTLSLTCAISGDSVSSNSAAWNWIRQSPSRGLEWLGRTYYRSKWYNDYAVSVKSRITINPDTSKNQFSLQLNSVTPEDTAVYYCAREGDDALDIWGQGTMVTVSSGGGGSGGGGSGGGGSDIQMTQSPSSLSASVGDRVTITCRASQSISHFLNWYQQKPGTAPKLLITTASGLGSGVPSRFSGSGSGTDFTLTINSLQPEDLATYYCQQSYTTPLTFGGGTKLEIKR

SEQ ID NO: 43 - DNA, 1470 bp, synthetic construct
  misc_feature 1..1470: note = Description of Artificial Sequence: Synthetic polynucleotide
  source 1..1470: mol_type = other DNA
atgcttctcctggtgacaagccttctgctctgtgagttaccacacccagcattcctcctgatcccacaagttcagttgcagcagagtggccctgggcttgttaaaccatcacagacgctctcactgacctgtgccatctctggagacagtgtaagttctaactcagccgcgtggaattggattagacaatcaccaagccggggacttgaatggcttggtcggacgtactatagatctaagtggtataatgactacgcagtgtcagtgaaatcacggataaccataaaccctgacaccagcaaaaaccaattttctcttcagcttaattccgtcacgccagaagatacggccgtttactactgtgcgagggaaggtgatgacgcattggacatctggggtcaggggaccatggtgactgtctcttccggcggggggggtagtggagggggtggctcaggtggtggcgggtcagatatacaaatgacacagagccctagtagtctgagtgcttcagtgggcgaccgcgtaactataacctgtagagcatcccaaagcatttcccacttccttaattggtaccagcagaagccgggcacagcgcccaaactcctgatcaccactgcgagcggacttggttcaggtgttcctagccggtttagtgggtcaggtagcggtacagatttcactctcacgataaactcccttcagcctgaggacctggcgacatattactgtcaacaatcctataccaccccactgacattcggagggggcacaaaactggagatcaaagcggccgcaactaccacccctgcccctcggccgccgactccggccccaaccatcgcaagccaacccctctccttgcgccccgaagcttgccgcccggccgcgggtggagccgtgcatacccgggggctggactttgcctgcgatatctacatttgggccccgctggccggcacttgcggcgtgctcctgctgtcgctggtcatcaccctttactgcaagaggggccggaagaagctgctttacatcttcaagcagccgttcatgcggcccgtgcagacgactcaggaagaggacggatgctcgtgcagattccctgaggaggaagaggggggatgcgaactgcgcgtcaagttctcacggtccgccgacgcccccgcatatcaacagggccagaatcagctctacaacgagctgaacctgggaaggagagaggagtacgacgtgctggacaagcgacgcggacgcgacccggagatgggggggaaaccacggcggaaaaaccctcaggaaggactgtacaacgaactccagaaagacaagatggcggaagcctactcagaaatcgggatgaagggagagcggaggaggggaaagggtcacgacgggctgtaccagggactgagcaccgccactaaggatacctacgatgccttgcatatgcaagcactcccaccccgg

SEQ ID NO: 44 - protein, 490 aa, synthetic construct
  REGION 1..490: note = Description of Artificial Sequence: Synthetic polypeptide
MLLLVTSLLLCELPHPAFLLIPQVQLQQSGPGLVKPSQTLSLTCAISGDSVSSNSAAWNWIRQSPSRGLEWLGRTYYRSKWYNDYAVSVKSRITINPDTSKNQFSLQLNSVTPEDTAVYYCAREGDDALDIWGQGTMVTVSSGGGGSGGGGSGGGGSDIQMTQSPSSLSASVGDRVTITCRASQSISHFLNWYQQKPGTAPKLLITTASGLGSGVPSRFSGSGSGTDFTLTINSLQPEDLATYYCQQSYTTPLTFGGGTKLEIKAAATTTPAPRPPTPAPTIASQPLSLRPEACRPAAGGAVHTRGLDFACDIYIWAPLAGTCGVLLLSLVITLYCKRGRKKLLYIFKQPFMRPVQTTQEEDGCSCRFPEEEEGGCELRVKFSRSADAPAYQQGQNQLYNELNLGRREEYDVLDKRRGRDPEMGGKPRRKNPQEGLYNELQKDKMAEAYSEIGMKGERRRGKGHDGLYQGLSTATKDTYDALHMQALPPR

SEQ ID NO: 45 - protein, 6 aa, synthetic construct
  REGION 1..6: note = Description of Artificial Sequence: Synthetic peptide
QSISHF

SEQ ID NO: 46 - skipped

SEQ ID NO: 47 - protein, 9 aa, synthetic construct
  REGION 1..9: note = Description of Artificial Sequence: Synthetic peptide
QQSYTTPLT

SEQ ID NO: 48 - protein, 10 aa, synthetic construct
  REGION 1..10: note = Description of Artificial Sequence: Synthetic peptide
GDSVSSNSAA

SEQ ID NO: 49 - protein, 9 aa, synthetic construct
  REGION 1..9: note = Description of Artificial Sequence: Synthetic peptide
TYYRSKWYN

SEQ ID NO: 50 - protein, 10 aa, synthetic construct
  REGION 1..10: note = Description of Artificial Sequence: Synthetic peptide
AREGDDALDI

SEQ ID NO: 51 - DNA, 732 bp, synthetic construct
  misc_feature 1..732: note = Description of Artificial Sequence: Synthetic polynucleotide
  source 1..732: mol_type = other DNA
cagatacagttgcagcagtcaggtccaggactagtgaagccctcgcagaccctctcactcacctgtgccatctccggggacagtgtctctagcaacagtgctgcttggaactggatcaggcagtccccatcgagaggccttgagtggctgggaaggacatactacaggtccaagtggtataatgattatgcagtatctgtgaaaagtcgaataaccatcaacccagacacatccaagaaccagttctccctgcagctgaactctgtgactcccgaggacacggctgtgtattactgtgcccaagaggtacaacctgatgatgctttagatatctggggccaagggacaatggtcaccgtctcttcaggaggtggcgggtctggcggtggaggtagcggtggtggcggatccgacatccagatgacccagtctccatcttccgtgtctgcatctgtaggagacaaagtcaccatcacttgtcgggcgagtcaggatgttagcggctggttagcctggtatcagcagaaaccagggctagcccctcagctcctgatctctggtgcatccactttgcaaggtgaagtcccatcaaggttcagcggcagtggatctgggacagattttactctcaccatcagcagcctgcagcctgaagattttgccacttattattgtcaacaggctaaaaatttcccttacacttttggccaggggaccaagctggaaatcaaa

SEQ ID NO: 52 - protein, 244 aa, synthetic construct
  REGION 1..244: note = Description of Artificial Sequence: Synthetic polypeptide
QIQLQQSGPGLVKPSQTLSLTCAISGDSVSSNSAAWNWIRQSPSRGLEWLGRTYYRSKWYNDYAVSVKSRITINPDTSKNQFSLQLNSVTPEDTAVYYCAQEVQPDDALDIWGQGTMVTVSSGGGGSGGGGSGGGGSDIQMTQSPSSVSASVGDKVTITCRASQDVSGWLAWYQQKPGLAPQLLISGASTLQGEVPSRFSGSGSGTDFTLTISSLQPEDFATYYCQQAKNFPYTFGQGTKLEIK

SEQ ID NO: 53 - DNA, 1476 bp, synthetic construct
  misc_feature 1..1476: note = Description of Artificial Sequence: Synthetic polynucleotide
  source 1..1476: mol_type = other DNA
atgttgttgcttgtcacaagccttcttctctgtgagcttccgcacccggctttcctgctgatcccgcagatacagcttcagcagtccggccccggtctggtaaagccgtcccaaacgctttcactcacatgcgcgatctctggtgattctgtgtcatccaacagcgcagcatggaattggatccgccaatcacccagtagaggcttggagtggttgggccggacttattatcgaagtaagtggtacaatgattatgcagtctcagttaaatccaggatcactattaacccagatacaagtaaaaaccagttctcattgcaacttaattccgtaactccggaggacactgcagtatattactgcgctcaggaggtgcagcctgatgatgctctggacatttggggacaaggcacgatggtcacggttagttccggggggggaggttctggcggaggtggtagtggggggggcggcagtgacatccagatgacacagagtcccagcagcgtgtctgcgtcagtcggggataaggtaacaattacgtgtagagcgagccaggacgtttccgggtggctggcgtggtaccaacaaaaacccggtctcgctccgcagttgctcatctctggagcgtccacccttcagggagaggtgcctagcagattttctgggtctggatccggcacggattttacacttacgatttcctctcttcaacccgaagattttgctacttactattgccagcaggccaaaaacttcccgtacacgtttggacagggcacaaagttggaaattaaggcggccgcaactaccacccctgcccctcggccgccgactccggccccaaccatcgcaagccaacccctctccttgcgccccgaagcttgccgcccggccgcgggtggagccgtgcatacccgggggctggactttgcctgcgatatctacatttgggccccgctggccggcacttgcggcgtgctcctgctgtcgctggtcatcaccctttactgcaagaggggccggaagaagctgctttacatcttcaagcagccgttcatgcggcccgtgcagacgactcaggaagaggacggatgctcgtgcagattccctgaggaggaagaggggggatgcgaactgcgcgtcaagttctcacggtccgccgacgcccccgcatatcaacagggccagaatcagctctacaacgagctgaacctgggaaggagagaggagtacgacgtgctggacaagcgacgcggacgcgacccggagatgggggggaaaccacggcggaaaaaccctcaggaaggactgtacaacgaactccagaaagacaagatggcggaagcctactcagaaatcgggatgaagggagagcggaggaggggaaagggtcacgacgggctgtaccagggactgagcaccgccactaaggatacctacgatgccttgcatatgcaagcactcccaccccgg

SEQ ID NO: 54 - protein, 492 aa, synthetic construct
  REGION 1..492: note = Description of Artificial Sequence: Synthetic polypeptide
MLLLVTSLLLCELPHPAFLLIPQIQLQQSGPGLVKPSQTLSLTCAISGDSVSSNSAAWNWIRQSPSRGLEWLGRTYYRSKWYNDYAVSVKSRITINPDTSKNQFSLQLNSVTPEDTAVYYCAQEVQPDDALDIWGQGTMVTVSSGGGGSGGGGSGGGGSDIQMTQSPSSVSASVGDKVTITCRASQDVSGWLAWYQQKPGLAPQLLISGASTLQGEVPSRFSGSGSGTDFTLTISSLQPEDFATYYCQQAKNFPYTFGQGTKLEIKAAATTTPAPRPPTPAPTIASQPLSLRPEACRPAAGGAVHTRGLDFACDIYIWAPLAGTCGVLLLSLVITLYCKRGRKKLLYIFKQPFMRPVQTTQEEDGCSCRFPEEEEGGCELRVKFSRSADAPAYQQGQNQLYNELNLGRREEYDVLDKRRGRDPEMGGKPRRKNPQEGLYNELQKDKMAEAYSEIGMKGERRRGKGHDGLYQGLSTATKDTYDALHMQALPPR

SEQ ID NO: 55 - protein, 6 aa, synthetic construct
  REGION 1..6: note = Description of Artificial Sequence: Synthetic peptide
QDVSGW

SEQ ID NO: 56 - skipped

SEQ ID NO: 57 - protein, 9 aa, synthetic construct
  REGION 1..9: note = Description of Artificial Sequence: Synthetic peptide
QQAKNFPYT

SEQ ID NO: 58 - protein, 10 aa, synthetic construct
  REGION 1..10: note = Description of Artificial Sequence: Synthetic peptide
GDSVSSNSAA

SEQ ID NO: 59 - protein, 9 aa, synthetic construct
  REGION 1..9: note = Description of Artificial Sequence: Synthetic peptide
TYYRSKWYN

SEQ ID NO: 60 - protein, 12 aa, synthetic construct
  REGION 1..12: note = Description of Artificial Sequence: Synthetic peptide
AQEVQPDDALDI

SEQ ID NO: 61 - DNA, 732 bp, synthetic construct
  misc_feature 1..732: note = Description of Artificial Sequence: Synthetic polynucleotide
  source 1..732: mol_type = other DNA
caagtacagttgcagcagtcaggacctggccttgtgaaaccatcccaaactctcagcctcacgtgtgctatttctggtgactcagtaagtagcaatagcgctgcttggaactggatcagacaatctccctccaggggtctcgaatggctggggcgaacctattaccgatctaaatggtataacgattatgcagtatccgtgaaatccaggattacaatcaacccagatacgttcaagaatcaattctctcttcagctcaactccgtaactccagaggacactgcggtatattattgcgcccaagaagtcgagccacacgatgccctcgatatctggggtcaaggtaccatggttacagttagtagtgggggtgggggaagcgggggcggtgggtccggtggcgggggttcagacatcaagatgacccaatccccaagctctgtttcagcatccgtgggcgataaggtaaccattacatgcagagcgagtcaggacgtttcagggtggctggcttggtaccagcaaaaaccgggactcgcaccgcagctgttgattttcggcgccagtacgcttcagggcgaagtaccgtccaggttcagtgggtcaggttctggcaccgattttacgctcacgatatccagtctccaaccggaggattttgctacttattactgccagcaggctaagtattttccatacacatttggccaggggacaaagttggagatcaaa

SEQ ID NO: 62 - protein, 244 aa, synthetic construct
  REGION 1..244: note = Description of Artificial Sequence: Synthetic polypeptide
QVQLQQSGPGLVKPSQTLSLTCAISGDSVSSNSAAWNWIRQSPSRGLEWLGRTYYRSKWYNDYAVSVKSRITINPDTFKNQFSLQLNSVTPEDTAVYYCAQEVEPHDALDIWGQGTMVTVSSGGGGSGGGGSGGGGSDIKMTQSPSSVSASVGDKVTITCRASQDVSGWLAWYQQKPGLAPQLLIFGASTLQGEVPSRFSGSGSGTDFTLTISSLQPEDFATYYCQQAKYFPYTFGQGTKLEIK

SEQ ID NO: 63 - DNA, 1476 bp, synthetic construct
  misc_feature 1..1476: note = Description of Artificial Sequence: Synthetic polynucleotide
  source 1..1476: mol_type = other DNA
atgctgcttttggtaacttccctccttttgtgcgagctgccccatccagcgttcctcctcatccctcaagtacagttgcagcagtcaggacctggccttgtgaaaccatcccaaactctcagcctcacgtgtgctatttctggtgactcagtaagtagcaatagcgctgcttggaactggatcagacaatctccctccaggggtctcgaatggctggggcgaacctattaccgatctaaatggtataacgattatgcagtatccgtgaaatccaggattacaatcaacccagatacgttcaagaatcaattctctcttcagctcaactccgtaactccagaggacactgcggtatattattgcgcccaagaagtcgagccacacgatgccctcgatatctggggtcaaggtaccatggttacagttagtagtgggggtgggggaagcgggggcggtgggtccggtggcgggggttcagacatcaagatgacccaatccccaagctctgtttcagcatccgtgggcgataaggtaaccattacatgcagagcgagtcaggacgtttcagggtggctggcttggtaccagcaaaaaccgggactcgcaccgcagctgttgattttcggcgccagtacgcttcagggcgaagtaccgtccaggttcagtgggtcaggttctggcaccgattttacgctcacgatatccagtctccaaccggaggattttgctacttattactgccagcaggctaagtattttccatacacatttggccaggggacaaagttggagatcaaagcggccgcaactaccacccctgcccctcggccgccgactccggccccaaccatcgcaagccaacccctctccttgcgccccgaagcttgccgcccggccgcgggtggagccgtgcatacccgggggctggactttgcctgcgatatctacatttgggccccgctggccggcacttgcggcgtgctcctgctgtcgctggtcatcaccctttactgcaagaggggccggaagaagctgctttacatcttcaagcagccgttcatgcggcccgtgcagacgactcaggaagaggacggatgctcgtgcagattccctgaggaggaagaggggggatgcgaactgcgcgtcaagttctcacggtccgccgacgcccccgcatatcaacagggccagaatcagctctacaacgagctgaacctgggaaggagagaggagtacgacgtgctggacaagcgacgcggacgcgacccggagatgggggggaaaccacggcggaaaaaccctcaggaaggactgtacaacgaactccagaaagacaagatggcggaagcctactcagaaatcgggatgaagggagagcggaggaggggaaagggtcacgacgggctgtaccagggactgagcaccgccactaaggatacctacgatgccttgcatatgcaagcactcccaccccgg

SEQ ID NO: 64 - protein, 492 aa, synthetic construct
  REGION 1..492: note = Description of Artificial Sequence: Synthetic polypeptide
MLLLVTSLLLCELPHPAFLLIPQVQLQQSGPGLVKPSQTLSLTCAISGDSVSSNSAAWNWIRQSPSRGLEWLGRTYYRSKWYNDYAVSVKSRITINPDTFKNQFSLQLNSVTPEDTAVYYCAQEVEPHDALDIWGQGTMVTVSSGGGGSGGGGSGGGGSDIKMTQSPSSVSASVGDKVTITCRASQDVSGWLAWYQQKPGLAPQLLIFGASTLQGEVPSRFSGSGSGTDFTLTISSLQPEDFATYYCQQAKYFPYTFGQGTKLEIKAAATTTPAPRPPTPAPTIASQPLSLRPEACRPAAGGAVHTRGLDFACDIYIWAPLAGTCGVLLLSLVITLYCKRGRKKLLYIFKQPFMRPVQTTQEEDGCSCRFPEEEEGGCELRVKFSRSADAPAYQQGQNQLYNELNLGRREEYDVLDKRRGRDPEMGGKPRRKNPQEGLYNELQKDKMAEAYSEIGMKGERRRGKGHDGLYQGLSTATKDTYDALHMQALPPR

SEQ ID NO: 65 - protein, 6 aa, synthetic construct
  REGION 1..6: note = Description of Artificial Sequence: Synthetic peptide
QDVSGW

SEQ ID NO: 66 - skipped

SEQ ID NO: 67 - protein, 9 aa, synthetic construct
  REGION 1..9: note = Description of Artificial Sequence: Synthetic peptide
QQAKYFPYT

SEQ ID NO: 68 - protein, 10 aa, synthetic construct
  REGION 1..10: note = Description of Artificial Sequence: Synthetic peptide
GDSVSSNSAA

SEQ ID NO: 69 - protein, 9 aa, synthetic construct
  REGION 1..9: note = Description of Artificial Sequence: Synthetic peptide
TYYRSKWYN

SEQ ID NO: 70 - protein, 12 aa, synthetic construct
  REGION 1..12: note = Description of Artificial Sequence: Synthetic peptide
AQEVEPHDALDI

SEQ ID NO: 71 - DNA, 732 bp, synthetic construct
  misc_feature 1..732: note = Description of Artificial Sequence: Synthetic polynucleotide
  source 1..732: mol_type = other DNA
caggtacagctgcagcagtcaggtccaggactggtgaagccctcgcagaccctctcactcacctgtgccatctccggggacagtgtctctagcaacagtgctgcttggaactggatcaggcagtccccatcgagaggccttgagtggctgggaaggacatactacaggtccaagtggtataatgattatgcagtatctgtgaaaagtcgaataaccatcaacccagacacatccaagaaccagttctccctgcagctgaactctgtgactcccgaggacacggctgtgtattactgtgcccaagaggtagaacctcatgatgctcttgatatctggggccaagggacaatggtcaccgtctcttcaggaggtggcgggtctggcggaggcggtagcggtggtggcggatccgacatccagatgacgcagtctccatcatccgtgtctgcatctgtaggagacaaagtcaccatcacttgtcgggcgagtcaggatgttagcggctggttagcctggtatcaacagaaaccagggctagcccctcagctcctgatctttggtgcatccactttgcaaggtgaagtcccatcaaggttcagcggcagtggatctgggacagattttactctcaccatcagcagcctgcagcctgaagattttgccacttattattgtcaacaggctaaatatttcccttacacttttggccaggggaccaagctggagatcaaa

SEQ ID NO: 72 - protein, 244 aa, synthetic construct
  REGION 1..244: note = Description of Artificial Sequence: Synthetic polypeptide
QVQLQQSGPGLVKPSQTLSLTCAISGDSVSSNSAAWNWIRQSPSRGLEWLGRTYYRSKWYNDYAVSVKSRITINPDTSKNQFSLQLNSVTPEDTAVYYCAQEVEPHDALDIWGQGTMVTVSSGGGGSGGGGSGGGGSDIQMTQSPSSVSASVGDKVTITCRASQDVSGWLAWYQQKPGLAPQLLIFGASTLQGEVPSRFSGSGSGTDFTLTISSLQPEDFATYYCQQAKYFPYTFGQGTKLEIK

SEQ ID NO: 73 - DNA, 1476 bp, synthetic construct
  misc_feature 1..1476: note = Description of Artificial Sequence: Synthetic polynucleotide
  source 1..1476: mol_type = other DNA
atgctgctcctcgtaacctctcttcttctttgtgagttgccacatccagcatttcttctgatacctcaagttcaactccagcagagtggtccaggtttggtaaaacccagccagactctctcattgacgtgtgccatatcaggtgattcagtttcctctaatagcgcggcatggaattggatcaggcaaagccctagtcgcgggctggagtggctcggccggacatactaccgctcaaagtggtacaacgactacgccgtcagcgtaaaatctcggattaccattaacccggatacttccaaaaaccaattctccctgcagcttaacagtgtcacgccggaagatacggccgtttattactgcgcacaagaggtggaaccgcacgacgccctcgatatctggggccaaggcactatggtgaccgtcagtagcggaggggggggttccggaggaggcggctctggtggcggaggatctgatatccaaatgacccaatcaccgtcttcagtatcagcttctgttggtgacaaagttacgattacctgtcgagcgtcacaggacgtttctggttggttggcttggtatcagcaaaaaccagggcttgcgcctcagttgcttatttttggggcatctactttgcagggagaggtgccctcccggttctccggcagtgggagcggcaccgattttacacttaccatctcttccttgcaacccgaagactttgcgacgtactattgccagcaggcaaagtattttccctacacttttggacaagggactaaacttgaaatcaaggcggccgcaactaccacccctgcccctcggccgccgactccggccccaaccatcgcaagccaacccctctccttgcgccccgaagcttgccgcccggccgcgggtggagccgtgcatacccgggggctggactttgcctgcgatatctacatttgggccccgctggccggcacttgcggcgtgctcctgctgtcgctggtcatcaccctttactgcaagaggggccggaagaagctgctttacatcttcaagcagccgttcatgcggcccgtgcagacgactcaggaagaggacggatgctcgtgcagattccctgaggaggaagaggggggatgcgaactgcgcgtcaagttctcacggtccgccgacgcccccgcatatcaacagggccagaatcagctctacaacgagctgaacctgggaaggagagaggagtacgacgtgctggacaagcgacgcggacgcgacccggagatgggggggaaaccacggcggaaaaaccctcaggaaggactgtacaacgaactccagaaagacaagatggcggaagcctactcagaaatcgggatgaagggagagcggaggaggggaaagggtcacgacgggctgtaccagggactgagcaccgccactaaggatacctacgatgccttgcatatgcaagcactcccaccccgg

SEQ ID NO: 74 - protein, 492 aa, synthetic construct
  REGION 1..492: note = Description of Artificial Sequence: Synthetic polypeptide
MLLLVTSLLLCELPHPAFLLIPQVQLQQSGPGLVKPSQTLSLTCAISGDSVSSNSAAWNWIRQSPSRGLEWLGRTYYRSKWYNDYAVSVKSRITINPDTSKNQFSLQLNSVTPEDTAVYYCAQEVEPHDALDIWGQGTMVTVSSGGGGSGGGGSGGGGSDIQMTQSPSSVSASVGDKVTITCRASQDVSGWLAWYQQKPGLAPQLLIFGASTLQGEVPSRFSGSGSGTDFTLTISSLQPEDFATYYCQQAKYFPYTFGQGTKLEIKAAATTTPAPRPPTPAPTIASQPLSLRPEACRPAAGGAVHTRGLDFACDIYIWAPLAGTCGVLLLSLVITLYCKRGRKKLLYIFKQPFMRPVQTTQEEDGCSCRFPEEEEGGCELRVKFSRSADAPAYQQGQNQLYNELNLGRREEYDVLDKRRGRDPEMGGKPRRKNPQEGLYNELQKDKMAEAYSEIGMKGERRRGKGHDGLYQGLSTATKDTYDALHMQALPPR

SEQ ID NO: 75 - protein, 6 aa, synthetic construct
  REGION 1..6: note = Description of Artificial Sequence: Synthetic peptide
QDVSGW

SEQ ID NO: 76 - skipped

SEQ ID NO: 77 - protein, 9 aa, synthetic construct
  REGION 1..9: note = Description of Artificial Sequence: Synthetic peptide
QQAKYFPYT

SEQ ID NO: 78 - protein, 10 aa, synthetic construct
  REGION 1..10: note = Description of Artificial Sequence: Synthetic peptide
GDSVSSNSAA

SEQ ID NO: 79 - protein, 9 aa, synthetic construct
  REGION 1..9: note = Description of Artificial Sequence: Synthetic peptide
TYYRSKWYN

SEQ ID NO: 80 - protein, 12 aa, synthetic construct
  REGION 1..12: note = Description of Artificial Sequence: Synthetic peptide
AQEVEPHDALDI

SEQ ID NO: 81 - DNA, 732 bp, synthetic construct
  misc_feature 1..732: note = Description of Artificial Sequence: Synthetic polynucleotide
  source 1..732: mol_type = other DNA
caggtacagctgcagcagtcaggtccaggactggtgaagccctcgcagaccctctcactcacctgtgccatctccggggacagtgtctctagcaacagtgctgcttggaactggatcaggcagtccccatcgagaggccttgagtggctgggaaggacatactacaggtccaagtggtataatgattatgcagtatctgtgaaaagtcgaataaccatcaacccagacacattcaagaaccagttctccctgcagctgaactctgtgactcccgaggacacggctgtgtattactgtgcccaagaggtagaacctcatgatgctcttgatatctggggccaagggacaatggtcaccgtctcttcaggaggtggcgggtctggcggtggaggtagcggtggtggcggatccgacatcaagatgacccagtctccatcttccgtgtctgcatctgtaggagacaaagtcaccatcacttgtcgggcgagtcaggatgttagcggctggttagcctggtatcagcagaaaccagggctagcccctcagctcctgatctttggtgcatccactttgcaaggtgaagtcccatcaaggttcagcggcagtggatctgggacagattttactctcaccatcagcagcctgcagcctgaagattttgccacttattattgtcaacaggctaaatatttcccttacacttttggccaggggaccaagctggaaatcaaa

SEQ ID NO: 82 - protein, 244 aa, synthetic construct; identical to SEQ ID NO: 62
  REGION 1..244: note = Description of Artificial Sequence: Synthetic polypeptide

SEQ ID NO: 83 - DNA, 1476 bp, synthetic construct
  misc_feature 1..1476: note = Description of Artificial Sequence: Synthetic polynucleotide
  source 1..1476: mol_type = other DNA
atgcttcttttggtgacttcccttttgctgtgcgagttgccacaccccgccttcctgcttattccccaagtccagctccaacaatccggacccggacttgttaagccgtctcagacgttgtcactcacatgcgccatcagtggcgatagcgtgtccagcaacagtgccgcatggaattggatacgacagagcccttcccgaggattggaatggctgggacgaacgtactataggtccaagtggtataacgactacgcggtgtcagttaaatctcggattactataaatcccgacacttttaagaatcagttttccctgcaactcaattcagtcacaccggaagatacggcagtgtactattgcgctcaagaagttgagccacatgatgcgctggatatttggggtcaggggactatggtgacggtaagcagtgggggcgggggcagtggcggaggtggcagcgggggcggtggaagcgacattaagatgactcagtctccgtcttcagtttccgcctccgtaggggacaaggttacaattacttgtcgcgcatctcaggatgtctcaggttggctggcttggtatcaacagaagcctggcctcgcccctcagcttctcatattcggggctagtaccctgcaaggagaagtcccgagcaggttttccggttcagggtccgggacagactttaccttgaccatcagctccctgcaaccggaggacttcgcgacctactattgtcaacaggcgaagtacttcccctacacgttcgggcaagggactaagctcgaaatcaaggcggccgcaactaccacccctgcccctcggccgccgactccggccccaaccatcgcaagccaacccctctccttgcgccccgaagcttgccgcccggccgcgggtggagccgtgcatacccgggggctggactttgcctgcgatatctacatttgggccccgctggccggcacttgcggcgtgctcctgctgtcgctggtcatcaccctttactgcaagaggggccggaagaagctgctttacatcttcaagcagccgttcatgcggcccgtgcagacgactcaggaagaggacggatgctcgtgcagattccctgaggaggaagaggggggatgcgaactgcgcgtcaagttctcacggtccgccgacgcccccgcatatcaacagggccagaatcagctctacaacgagctgaacctgggaaggagagaggagtacgacgtgctggacaagcgacgcggacgcgacccggagatgggggggaaaccacggcggaaaaaccctcaggaaggactgtacaacgaactccagaaagacaagatggcggaagcctactcagaaatcgggatgaagggagagcggaggaggggaaagggtcacgacgggctgtaccagggactgagcaccgccactaaggatacctacgatgccttgcatatgcaagcactcccaccccgg

SEQ ID NO: 84 - protein, 492 aa, synthetic construct; identical to SEQ ID NO: 64
  REGION 1..492: note = Description of Artificial Sequence: Synthetic polypeptide

SEQ ID NO: 85 - protein, 6 aa, synthetic construct
  REGION 1..6: note = Description of Artificial Sequence: Synthetic peptide
QDVSGW

SEQ ID NO: 86 - skipped

SEQ ID NO: 87 - protein, 9 aa, synthetic construct
  REGION 1..9: note = Description of Artificial Sequence: Synthetic peptide
QQAKYFPYT

SEQ ID NO: 88 - protein, 10 aa, synthetic construct
  REGION 1..10: note = Description of Artificial Sequence: Synthetic peptide
GDSVSSNSAA

SEQ ID NO: 89 - protein, 9 aa, synthetic construct
  REGION 1..9: note = Description of Artificial Sequence: Synthetic peptide
TYYRSKWYN

SEQ ID NO: 90 - protein, 12 aa, synthetic construct
  REGION 1..12: note = Description of Artificial Sequence: Synthetic peptide
AQEVEPHDALDI

SEQ ID NO: 91 - DNA, 732 bp, synthetic construct
  misc_feature 1..732: note = Description of Artificial Sequence: Synthetic polynucleotide
  source 1..732: mol_type = other DNA
caggtacagctgcagcagtcaggtccaggactggtgaagccctcgcagaccctctcactcacctgtgccatctccggggacagtgtctctagcaacagtgctgcttggaactggatcaggcagtccccatcgagaggccttgagtggctgggaaggacatactacaggtccaagtggtataatgattatgcagtatctgtgaaaagtcgaataaccatcaacccagacacatccaagaaccagttctccctgcagctgaactctgtgactcccgaggatacggctgtgtattactgtgcccaagaggtacaacctgatgatgcttttgatatctggggccaagggacaatgatcaccgtctcttcaggaggtggcgggtctggcggtggaggtagcggtggtggcggatccgacatccagatgacccagtctccatcttccgtgtctgcatctgtaggagacaaagtcaccatcacttgtcgggcgagtcaggatgttagcggctggttagcctggtatcagcagaaaccagggctagcccctcagctcctgatctctggtgcatccactttgcaaggtggagtcccatcaaggttcagcggcagtggatctgggacagattttactctcaccatcagcagcctgcagcctgaagattttgccacttattattgtcaacaggctaaaaatttcccttacacttttggtcaggggaccaagctggaaatcaaa

SEQ ID NO: 92 - protein, 244 aa, synthetic construct
  REGION 1..244: note = Description of Artificial Sequence: Synthetic polypeptide
QVQLQQSGPGLVKPSQTLSLTCAISGDSVSSNSAAWNWIRQSPSRGLEWLGRTYYRSKWYNDYAVSVKSRITINPDTSKNQFSLQLNSVTPEDTAVYYCAQEVQPDDAFDIWGQGTMITVSSGGGGSGGGGSGGGGSDIQMTQSPSSVSASVGDKVTITCRASQDVSGWLAWYQQKPGLAPQLLISGASTLQGGVPSRFSGSGSGTDFTLTISSLQPEDFATYYCQQAKNFPYTFGQGTKLEIK

SEQ ID NO: 93 - DNA, 1476 bp, synthetic construct
  misc_feature 1..1476: note = Description of Artificial Sequence: Synthetic polynucleotide
  source 1..1476: mol_type = other DNA
atgcttcttttggtgacttcccttttgctgtgcgagttgccacaccccgccttcctgcttattccccaagtacaactccagcaatcagggcctggccttgtcaagccgagtcaaaccttgagtttgacgtgtgccatcagcggtgactctgtcagttcaaactccgcagcttggaactggattcggcagtccccctccaggggcctcgaatggcttggacggacgtactacagatcaaaatggtacaacgactacgcagtcagtgtaaaatcaaggattacgataaaccctgatacgagtaaaaaccagttctctctccaactgaacagcgtcacaccggaagatacagccgtgtattactgtgctcaggaagtgcaacctgacgacgcatttgacatctggggtcagggcacgatgatcaccgtgagtagtggaggaggaggcagtgggggaggcggttctggcgggggtgggtctgatatacagatgacacagagtccctcctcagtttccgcctctgttggagataaggtgacaattacatgcagggcgtcccaagatgtttctggatggctcgcatggtaccaacagaagccaggactcgcccctcagctcctcattagcggcgctagcactctccaagggggagtaccgagcaggttctctgggtccggaagtgggacggactttaccctgacaatatcctcccttcagccagaagacttcgcaacctactattgccaacaggcgaaaaatttcccttacacgttcggccaaggaactaaacttgaaatcaaggcggccgcaactaccacccctgcccctcggccgccgactccggccccaaccatcgcaagccaacccctctccttgcgccccgaagcttgccgcccggccgcgggtggagccgtgcatacccgggggctggactttgcctgcgatatctacatttgggccccgctggccggcacttgcggcgtgctcctgctgtcgctggtcatcaccctttactgcaagaggggccggaagaagctgctttacatcttcaagcagccgttcatgcggcccgtgcagacgactcaggaagaggacggatgctcgtgcagattccctgaggaggaagaggggggatgcgaactgcgcgtcaagttctcacggtccgccgacgcccccgcatatcaacagggccagaatcagctctacaacgagctgaacctgggaaggagagaggagtacgacgtgctggacaagcgacgcggacgcgacccggagatgggggggaaaccacggcggaaaaaccctcaggaaggactgtacaacgaactccagaaagacaagatggcggaagcctactcagaaatcgggatgaagggagagcggaggaggggaaagggtcacgacgggctgtaccagggactgagcaccgccactaaggatacctacgatgccttgcatatgcaagcactcccaccccgg

SEQ ID NO: 94 - protein, 492 aa, synthetic construct
  REGION 1..492: note = Description of Artificial Sequence: Synthetic polypeptide
MLLLVTSLLLCELPHPAFLLIPQVQLQQSGPGLVKPSQTLSLTCAISGDSVSSNSAAWNWIRQSPSRGLEWLGRTYYRSKWYNDYAVSVKSRITINPDTSKNQFSLQLNSVTPEDTAVYYCAQEVQPDDAFDIWGQGTMITVSSGGGGSGGGGSGGGGSDIQMTQSPSSVSASVGDKVTITCRASQDVSGWLAWYQQKPGLAPQLLISGASTLQGGVPSRFSGSGSGTDFTLTISSLQPEDFATYYCQQAKNFPYTFGQGTKLEIKAAATTTPAPRPPTPAPTIASQPLSLRPEACRPAAGGAVHTRGLDFACDIYIWAPLAGTCGVLLLSLVITLYCKRGRKKLLYIFKQPFMRPVQTTQEEDGCSCRFPEEEEGGCELRVKFSRSADAPAYQQGQNQLYNELNLGRREEYDVLDKRRGRDPEMGGKPRRKNPQEGLYNELQKDKMAEAYSEIGMKGERRRGKGHDGLYQGLSTATKDTYDALHMQALPPR

SEQ ID NO: 95 - protein, 6 aa, synthetic construct
  REGION 1..6: note = Description of Artificial Sequence: Synthetic peptide
QDVSGW

SEQ ID NO: 96 - skipped

SEQ ID NO: 97 - protein, 9 aa, synthetic construct
  REGION 1..9: note = Description of Artificial Sequence: Synthetic peptide
QQAKNFPYT

SEQ ID NO: 98 - protein, 10 aa, synthetic construct
  REGION 1..10: note = Description of Artificial Sequence: Synthetic peptide
GDSVSSNSAA

SEQ ID NO: 99 - protein, 9 aa, synthetic construct
  REGION 1..9: note = Description of Artificial Sequence: Synthetic peptide
TYYRSKWYN

SEQ ID NO: 100 - protein, 12 aa, synthetic construct
  REGION 1..12: note = Description of Artificial Sequence: Synthetic peptide
AQEVQPDDAFDI

SEQ ID NO: 101 - DNA, 732 bp, synthetic construct
  misc_feature 1..732: note = Description of Artificial Sequence: Synthetic polynucleotide
  source 1..732: mol_type = other DNA
caggtacagctgcagcagtcaggtccaggactggtgaagccctcgcagaccctctcactcacctgtgccatctccggggacagtgtctctagcaacagtgctgcttggaactggatcaggcagtccccatcgagaggccttgagtggctgggaaggacatactacaggtccaagtggtataatgattatgcagtatctgtgaaaagtcgaataaccatcaacccagacacatccaagaaccagttctccctgcagctgaactctgtgactcccgaggacacggctgtgtattactgtgcccaagaggtagaacctcaggatgcttttgatatctggggccaagggacaatggtcaccgtctcttcaggaggtggcgggtctggtggtggcggtagcggtggtggcggatccgacatccagatgacccagtctccatcttccgtgtctgcatctgtaggagacaaagtcaccatcacttgtcgggcgagtcaggatgttagcggctggttagcctggtatcagcagaaaccagggctagcccctcagctcctgatctttggtgcatccactctgcaaggtgaagtcccatcaaggttcagtggcagtggatctgggacagattttactctcaccatcagcagcctgcagcctgaagattttgccacttattattgtcaacaggctaaatatttcccttacacttttggcccggggaccaagctggaaatcaaa

SEQ ID NO: 102 - protein, 244 aa, synthetic construct
  REGION 1..244: note = Description of Artificial Sequence: Synthetic polypeptide
QVQLQQSGPGLVKPSQTLSLTCAISGDSVSSNSAAWNWIRQSPSRGLEWLGRTYYRSKWYNDYAVSVKSRITINPDTSKNQFSLQLNSVTPEDTAVYYCAQEVEPQDAFDIWGQGTMVTVSSGGGGSGGGGSGGGGSDIQMTQSPSSVSASVGDKVTITCRASQDVSGWLAWYQQKPGLAPQLLIFGASTLQGEVPSRFSGSGSGTDFTLTISSLQPEDFATYYCQQAKYFPYTFGPGTKLEIK

SEQ ID NO: 103 - DNA, 1476 bp, synthetic construct
  misc_feature 1..1476: note = Description of Artificial Sequence: Synthetic polynucleotide
  source 1..1476: mol_type = other DNA
atgcttcttttggtgacttcccttttgctgtgcgagttgccacaccccgccttcctgcttattccccaagtgcagttgcaacagtctggaccaggcctcgtaaaaccttctcaaactttgtcactcacttgtgccatctcaggggacagtgtcagttccaacagtgcggcatggaattggattaggcaatccccctctcgaggtctggaatggcttgggcggacttactaccgaagtaagtggtacaacgattatgcagtttctgtaaaatcacgaatcactataaatccggacacttctaagaatcagttctctttgcagcttaactctgttactcctgaagacacagccgtatattactgtgctcaagaggtagagccgcaagatgccttcgacatctggggccaagggactatggtgacagtaagctccggaggtgggggatcagggggaggtgggtccggtggtggtggctctgacatacagatgacacagtcccctagctctgtgtcagcaagtgtcggtgacaaggttacgataacgtgcagggccagtcaagatgtgtcaggatggttggcgtggtaccaacagaaacccggcttggcaccgcagcttttgatattcggcgcgtccacactccaaggcgaagtgccttctcggttttctggaagcggcagcgggacggactttactttgacaatatcctccctccaacccgaggatttcgcgacgtattattgccagcaagcaaaatacttcccatacaccttcgggcctgggaccaaactggagatcaaagcggccgcaactaccacccctgcccctcggccgccgactccggccccaaccatcgcaagccaacccctctccttgcgccccgaagcttgccgcccggccgcgggtggagccgtgcatacccgggggctggactttgcctgcgatatctacatttgggccccgctggccggcacttgcggcgtgctcctgctgtcgctggtcatcaccctttactgcaagaggggccggaagaagctgctttacatcttcaagcagccgttcatgcggcccgtgcagacgactcaggaagaggacggatgctcgtgcagattccctgaggaggaagaggggggatgcgaactgcgcgtcaagttctcacggtccgccgacgcccccgcatatcaacagggccagaatcagctctacaacgagctgaacctgggaaggagagaggagtacgacgtgctggacaagcgacgcggacgcgacccggagatgggggggaaaccacggcggaaaaaccctcaggaaggactgtacaacgaactccagaaagacaagatggcggaagcctactcagaaatcgggatgaagggagagcggaggaggggaaagggtcacgacgggctgtaccagggactgagcaccgccactaaggatacctacgatgccttgcatatgcaagcactcccaccccgg

SEQ ID NO: 104 - protein, 492 aa, synthetic construct
  REGION 1..492: note = Description of Artificial Sequence: Synthetic polypeptide
MLLLVTSLLLCELPHPAFLLIPQVQLQQSGPGLVKPSQTLSLTCAISGDSVSSNSAAWNWIRQSPSRGLEWLGRTYYRSKWYNDYAVSVKSRITINPDTSKNQFSLQLNSVTPEDTAVYYCAQEVEPQDAFDIWGQGTMVTVSSGGGGSGGGGSGGGGSDIQMTQSPSSVSASVGDKVTITCRASQDVSGWLAWYQQKPGLAPQLLIFGASTLQGEVPSRFSGSGSGTDFTLTISSLQPEDFATYYCQQAKYFPYTFGPGTKLEIKAAATTTPAPRPPTPAPTIASQPLSLRPEACRPAAGGAVHTRGLDFACDIYIWAPLAGTCGVLLLSLVITLYCKRGRKKLLYIFKQPFMRPVQTTQEEDGCSCRFPEEEEGGCELRVKFSRSADAPAYQQGQNQLYNELNLGRREEYDVLDKRRGRDPEMGGKPRRKNPQEGLYNELQKDKMAEAYSEIGMKGERRRGKGHDGLYQGLSTATKDTYDALHMQALPPR

SEQ ID NO: 105 - protein, 6 aa, synthetic construct
  REGION 1..6: note = Description of Artificial Sequence: Synthetic peptide
QDVSGW

SEQ ID NO: 106 - skipped

SEQ ID NO: 107 - protein, 9 aa, synthetic construct
  REGION 1..9: note = Description of Artificial Sequence: Synthetic peptide
QQAKYFPYT

SEQ ID NO: 108 - protein, 10 aa, synthetic construct
  REGION 1..10: note = Description of Artificial Sequence: Synthetic peptide
GDSVSSNSAA

SEQ ID NO: 109 - protein, 9 aa, synthetic construct
  REGION 1..9: note = Description of Artificial Sequence: Synthetic peptide
TYYRSKWYN

SEQ ID NO: 110 - protein, 12 aa, synthetic construct
  REGION 1..12: note = Description of Artificial Sequence: Synthetic peptide
AQEVEPQDAFDI

SEQ ID NO: 111 - DNA, 732 bp, synthetic construct
  misc_feature 1..732: note = Description of Artificial Sequence: Synthetic polynucleotide
  source 1..732: mol_type = other DNA
caggtacagctgcagcagtcaggtccaggactggtgaagcactcgcagaccctctcactcacctgtgccatctccggggacagtgtctctagcaacagtgctgcttggaactggatcaggcagtccccatcgagaggccttgagtggctgggaaggacatactacaggtccaagtggtataatgattatgcagtatctgtgaaaagtcgaataaccatcaacccagacacatccaagaaccagttctccctgcagttgaactctgtgactcccgaggacacggctgtgtattactgtgcccaagaggtagaacctcatgatgcttttgatatctggggccaagggacaatggtcaccgtctcttcaggaggtggcgggtctggcggtggaggtagcggtggtggcggatccgacatccagatgacccagtctccatcttccgtgtatgcatctgtaggagacaaagtcaccatcacttgtcgggcgagtcaggatgttagcggctggttagcctggtatcagcagaaaccagggctagcccctcagctcctgatctctggtgcatccactttgcaaggtgaagtcccatcaaggttcagcggcagtggatctgggacagattttactctcaccatcagcagcctgcagcctgaagattttgccacttattattgtcaacaggctaaatatttcccttacacttttggccaggggaccaagctggaaatcaaa

SEQ ID NO: 112 - protein, 244 aa, synthetic construct
  REGION 1..244: note = Description of Artificial Sequence: Synthetic polypeptide
QVQLQQSGPGLVKHSQTLSLTCAISGDSVSSNSAAWNWIRQSPSRGLEWLGRTYYRSKWYNDYAVSVKSRITINPDTSKNQFSLQLNSVTPEDTAVYYCAQEVEPHDAFDIWGQGTMVTVSSGGGGSGGGGSGGGGSDIQMTQSPSSVYASVGDKVTITCRASQDVSGWLAWYQQKPGLAPQLLISGASTLQGEVPSRFSGSGSGTDFTLTISSLQPEDFATYYCQQAKYFPYTFGQGTKLEIK

SEQ ID NO: 113 - DNA, 1476 bp, synthetic construct
  misc_feature 1..1476: note = Description of Artificial Sequence: Synthetic polynucleotide
  source 1..1476: mol_type = other DNA
atgcttcttttggtgacttcccttttgctgtgcgagttgccacaccccgccttcctgcttattccccaggtacagcttcaacagagtgggccgggactggtgaaacactcccaaacactttctctgacgtgcgctatatcaggtgactctgtttcatctaattctgctgcgtggaactggattcgacaatctcccagtcgcgggttggaatggctgggacgaacatattatcggtctaagtggtataacgattatgctgtatctgttaaatctcgaattacgattaatcctgacacctccaagaaccagttctccctccagttgaactcagtcacaccggaagacactgcggtctactattgcgctcaagaagtcgagccacatgatgcattcgacatctggggccagggaacgatggtcaccgtcagcagtggcggcggcggatctgggggtggcggttctggcggtggaggatcagacatacaaatgacgcagagtccctcaagtgtgtacgcgagtgtgggggataaggtaactattacgtgcagagcgtcacaggatgttagtggatggcttgcctggtatcagcagaagccaggccttgctccacagctccttatcagtggtgcttctacacttcagggcgaggttccgagtagattctctggttctggatctggtactgacttcactcttacaatttcttctttgcaaccagaagactttgcgacttattactgccaacaggccaaatacttcccttatacatttggccaaggtaccaagttggagataaaggcggccgcaactaccacccctgcccctcggccgccgactccggccccaaccatcgcaagccaacccctctccttgcgccccgaagcttgccgcccggccgcgggtggagccgtgcatacccgggggctggactttgcctgcgatatctacatttgggccccgctggccggcacttgcggcgtgctcctgctgtcgctggtcatcaccctttactgcaagaggggccggaagaagctgctttacatcttcaagcagccgttcatgcggcccgtgcagacgactcaggaagaggacggatgctcgtgcagattccctgaggaggaagaggggggatgcgaactgcgcgtcaagttctcacggtccgccgacgcccccgcatatcaacagggccagaatcagctctacaacgagctgaacctgggaaggagagaggagtacgacgtgctggacaagcgacgcggacgcgacccggagatgggggggaaaccacggcggaaaaaccctcaggaaggactgtacaacgaactccagaaagacaagatggcggaagcctactcagaaatcgggatgaagggagagcggaggaggggaaagggtcacgacgggctgtaccagggactgagcaccgccactaaggatacctacgatgccttgcatatgcaagcactcccaccccgg

SEQ ID NO: 114 - protein, 492 aa, synthetic construct
  REGION 1..492: note = Description of Artificial Sequence: Synthetic polypeptide
MLLLVTSLLLCELPHPAFLLIPQVQLQQSGPGLVKHSQTLSLTCAISGDSVSSNSAAWNWIRQSPSRGLEWLGRTYYRSKWYNDYAVSVKSRITINPDTSKNQFSLQLNSVTPEDTAVYYCAQEVEPHDAFDIWGQGTMVTVSSGGGGSGGGGSGGGGSDIQMTQSPSSVYASVGDKVTITCRASQDVSGWLAWYQQKPGLAPQLLISGASTLQGEVPSRFSGSGSGTDFTLTISSLQPEDFATYYCQQAKYFPYTFGQGTKLEIKAAATTTPAPRPPTPAPTIASQPLSLRPEACRPAAGGAVHTRGLDFACDIYIWAPLAGTCGVLLLSLVITLYCKRGRKKLLYIFKQPFMRPVQTTQEEDGCSCRFPEEEEGGCELRVKFSRSADAPAYQQGQNQLYNELNLGRREEYDVLDKRRGRDPEMGGKPRRKNPQEGLYNELQKDKMAEAYSEIGMKGERRRGKGHDGLYQGLSTATKDTYDALHMQALPPR

SEQ ID NO: 115 - protein, 6 aa, synthetic construct
  REGION 1..6: note = Description of Artificial Sequence: Synthetic peptide
QDVSGW

SEQ ID NO: 116 - skipped

SEQ ID NO: 117 - protein, 9 aa, synthetic construct
  REGION 1..9: note = Description of Artificial Sequence: Synthetic peptide
QQAKYFPYT

SEQ ID NO: 118 - protein, 10 aa, synthetic construct
  REGION 1..10: note = Description of Artificial Sequence: Synthetic peptide
GDSVSSNSAA

SEQ ID NO: 119 - protein, 9 aa, synthetic construct
  REGION 1..9: note = Description of Artificial Sequence: Synthetic peptide
TYYRSKWYN

SEQ ID NO: 120 - protein, 12 aa, synthetic construct
  REGION 1..12: note = Description of Artificial Sequence: Synthetic peptide
AQEVEPHDAFDI

SEQ ID NO: 121 - DNA, 732 bp, synthetic construct
  misc_feature 1..732: note = Description of Artificial Sequence: Synthetic polynucleotide
  source 1..732: mol_type = other DNA
caagtacaacttcaacagtctgggcctgggcttgtaaaacctagccaaactctgtccctcacgtgcgcgatttcaggggacagtgtaagttccaactcagccgcatggaactggatcaggcagtcaccttcaagggggctcgaatggcttggccgaacgtactacaggagtaagtggtacaacgattatgcagtgtctgtgaaatcacggattactatcaatcccgacacgtccaagaaccagttctctctgcaactcaactcagtgacaccagaggatacggccgtttactattgtgcacaggaagtgcaacctgatgatgcctttgacatttggggtcagggcacgatggttacggtaagctctgggggaggcggcagtggagggggaggtagtgggggagggggatctgatatacagatgacacaaagcccgtcatccgtcagtgcttcagttggtgataaagtaaccattacgtgccgcgcttcccaagacgttagcggatggttggcttggtatcaacaaaaaccggggttggctccgcaactcctcatatccggtgcgagtacgctccaaggcgaagtccctagcagattttccgggagcggttccggtacagatttcacgttgaccattagctctctccagcccgaagattttgcaacctactattgccaacaggccaaaaattttccatatacatttggtcaaggcactaagctcgaaatcaaa

SEQ ID NO: 122 - protein, 244 aa, synthetic construct
  REGION 1..244: note = Description of Artificial Sequence: Synthetic polypeptide
QVQLQQSGPGLVKPSQTLSLTCAISGDSVSSNSAAWNWIRQSPSRGLEWLGRTYYRSKWYNDYAVSVKSRITINPDTSKNQFSLQLNSVTPEDTAVYYCAQEVQPDDAFDIWGQGTMVTVSSGGGGSGGGGSGGGGSDIQMTQSPSSVSASVGDKVTITCRASQDVSGWLAWYQQKPGLAPQLLISGASTLQGEVPSRFSGSGSGTDFTLTISSLQPEDFATYYCQQAKNFPYTFGQGTKLEIK

SEQ ID NO: 123 - DNA, 1476 bp, synthetic construct
  misc_feature 1..1476: note = Description of Artificial Sequence: Synthetic polynucleotide
  source 1..1476: mol_type = other DNA
atgcttcttttggtgacttcccttttgctgtgcgagttgccacaccccgccttcctgcttattccccaagtacaacttcaacagtctgggcctgggcttgtaaaacctagccaaactctgtccctcacgtgcgcgatttcaggggacagtgtaagttccaactcagccgcatggaactggatcaggcagtcaccttcaagggggctcgaatggcttggccgaacgtactacaggagtaagtggtacaacgattatgcagtgtctgtgaaatcacggattactatcaatcccgacacgtccaagaaccagttctctctgcaactcaactcagtgacaccagaggatacggccgtttactattgtgcacaggaagtgcaacctgatgatgcctttgacatttggggtcagggcacgatggttacggtaagctctgggggaggcggcagtggagggggaggtagtgggggagggggatctgatatacagatgacacaaagcccgtcatccgtcagtgcttcagttggtgataaagtaaccattacgtgccgcgcttcccaagacgttagcggatggttggcttggtatcaacaaaaaccggggttggctccgcaactcctcatatccggtgcgagtacgctccaaggcgaagtccctagcagattttccgggagcggttccggtacagatttcacgttgaccattagctctctccagcccgaagattttgcaacctactattgccaacaggccaaaaattttccatatacatttggtcaaggcactaagctcgaaatcaaagcggccgcaactaccacccctgcccctcggccgccgactccggccccaaccatcgcaagccaacccctctccttgcgccccgaagcttgccgcccggccgcgggtggagccgtgcatacccgggggctggactttgcctgcgatatctacatttgggccccgctggccggcacttgcggcgtgctcctgctgtcgctggtcatcaccctttactgcaagaggggccggaagaagctgctttacatcttcaagcagccgttcatgcggcccgtgcagacgactcaggaagaggacggatgctcgtgcagattccctgaggaggaagaggggggatgcgaactgcgcgtcaagttctcacggtccgccgacgcccccgcatatcaacagggccagaatcagctctacaacgagctgaacctgggaaggagagaggagtacgacgtgctggacaagcgacgcggacgcgacccggagatgggggggaaaccacggcggaaaaaccctcaggaaggactgtacaacgaactccagaaagacaagatggcggaagcctactcagaaatcgggatgaagggagagcggaggaggggaaagggtcacgacgggctgtaccagggactgagcaccgccactaaggatacctacgatgccttgcatatgcaagcactcccaccccgg

SEQ ID NO: 124 - protein, 492 aa, synthetic construct
  REGION 1..492: note = Description of Artificial Sequence: Synthetic polypeptide
MLLLVTSLLLCELPHPAFLLIPQVQLQQSGPGLVKPSQTLSLTCAISGDSVSSNSAAWNWIRQSPSRGLEWLGRTYYRSKWYNDYAVSVKSRITINPDTSKNQFSLQLNSVTPEDTAVYYCAQEVQPDDAFDIWGQGTMVTVSSGGGGSGGGGSGGGGSDIQMTQSPSSVSASVGDKVTITCRASQDVSGWLAWYQQKPGLAPQLLISGASTLQGEVPSRFSGSGSGTDFTLTISSLQPEDFATYYCQQAKNFPYTFGQGTKLEIKAAATTTPAPRPPTPAPTIASQPLSLRPEACRPAAGGAVHTRGLDFACDIYIWAPLAGTCGVLLLSLVITLYCKRGRKKLLYIFKQPFMRPVQTTQEEDGCSCRFPEEEEGGCELRVKFSRSADAPAYQQGQNQLYNELNLGRREEYDVLDKRRGRDPEMGGKPRRKNPQEGLYNELQKDKMAEAYSEIGMKGERRRGKGHDGLYQGLSTATKDTYDALHMQALPPR

SEQ ID NO: 125 - protein, 6 aa, synthetic construct
  REGION 1..6: note = Description of Artificial Sequence: Synthetic peptide
QDVSGW

SEQ ID NO: 126 - skipped

SEQ ID NO: 127 - protein, 9 aa, synthetic construct
  REGION 1..9: note = Description of Artificial Sequence: Synthetic peptide
QQAKNFPYT

SEQ ID NO: 128 - protein, 10 aa, synthetic construct
  REGION 1..10: note = Description of Artificial Sequence: Synthetic peptide
GDSVSSNSAA

SEQ ID NO: 129 - protein, 9 aa, synthetic construct
  REGION 1..9: note = Description of Artificial Sequence: Synthetic peptide
TYYRSKWYN

SEQ ID NO: 130 - protein, 12 aa, synthetic construct
  REGION 1..12: note = Description of Artificial Sequence: Synthetic peptide
AQEVQPDDAFDI

SEQ ID NO: 131 - DNA, 732 bp, synthetic construct
  misc_feature 1..732: note = Description of Artificial Sequence: Synthetic polynucleotide
  source 1..732: mol_type = other DNA
caggtacagctgcagcagtcaggtccaggactggtgaagccctcgcagaccctctcactcacctgtgacatctccggggacagtgtctctagcaacagtgctgcttggaactggatcaggcagtccccatcgagaggccttgagtggctgggaaggacatactacaggtccaagtggtataatgattatgcagtatctgtgaaaagtcgaataaccatcaacccagacacatccaagaaccagttctccctgcagctgaactctgtgactcccgaggacacggctgtgtattactgtgcccaagagatagaacctcatgatgcttttgatatctgggaccaagggacaatggtcaccgtctcttcaggaggtggcgggtctggcggtggaggtagcggtggtggcggatccgtcatccagatgacccagtctccatcttccgtgtctgcatctgtaggagacaaagtcaccatcacttgtcgggcgagtcaggatgttagcggctggttagcctggtatcagcagaaaccagggctagcccctcagctcctgatctctggtgcatcctctttgcaaggtggagtcccatcaaggttcagcggcagtggatctgggacagattttactctcaccatcagcagcctgcagcctgaagattttgccacttattattgtcaacaggctaaatatttcccttacacttttggccaggggaccaagctggaaatcaaa

SEQ ID NO: 132 - protein, 244 aa, synthetic construct
  REGION 1..244: note = Description of Artificial Sequence: Synthetic polypeptide
QVQLQQSGPGLVKPSQTLSLTCDISGDSVSSNSAAWNWIRQSPSRGLEWLGRTYYRSKWYNDYAVSVKSRITINPDTSKNQFSLQLNSVTPEDTAVYYCAQEIEPHDAFDIWDQGTMVTVSSGGGGSGGGGSGGGGSVIQMTQSPSSVSASVGDKVTITCRASQDVSGWLAWYQQKPGLAPQLLISGASSLQGGVPSRFSGSGSGTDFTLTISSLQPEDFATYYCQQAKYFPYTFGQGTKLEIK

SEQ ID NO: 133 - DNA, 1476 bp, synthetic construct
  misc_feature 1..1476: note = Description of Artificial Sequence: Synthetic polynucleotide
  source 1..1476: mol_type = other DNA
atgttgctgctcgtgacctcgctccttctgtgcgagctgccccatccggcttttctgctcatccctcaagtgcagctgcagcagtccggtcctggactggtcaagccgtcccagactctgagcctgacttgcgatattagcggggactcagtctcgtccaattcggcggcctggaactggatccggcagtcaccatcaaggggcctggaatggctcgggcgcacttactaccggtccaaatggtataacgactacgccgtgtccgtgaagtcccggatcaccattaaccccgacacctcgaagaaccagttctcactccaactgaacagcgtgacccccgaggataccgcggtgtactactgcgcacaagaaatcgaaccgcacgacgccttcgacatttgggaccagggaacgatggtcacagtgtcgtccggtggaggaggttccggaggcggtggatctggaggcggaggttcggtgatccagatgacccagagcccctcctcggtgtccgcatccgtgggcgataaggtcaccattacctgtagagcgtcccaggacgtgtccggatggctggcctggtaccagcagaagccaggcttggctcctcaactgctgatctccggcgccagctcacttcaggggggggtgccatcacgcttctccggatccggttccggcaccgacttcaccctgaccatcagcagcctccagcctgaggacttcgccacttactactgccaacaggccaagtacttcccctataccttcggacaaggcactaagctggaaatcaaggcggccgcaactaccacccctgcccctcggccgccgactccggccccaaccatcgcaagccaacccctctccttgcgccccgaagcttgccgcccggccgcgggtggagccgtgcatacccgggggctggactttgcctgcgatatctacatttgggccccgctggccggcacttgcggcgtgctcctgctgtcgctggtcatcaccctttactgcaagaggggccggaagaagctgctttacatcttcaagcagccgttcatgcggcccgtgcagacgactcaggaagaggacggatgctcgtgcagattccctgaggaggaagaggggggatgcgaactgcgcgtcaagttctcacggtccgccgacgcccccgcatatcaacagggccagaatcagctctacaacgagctgaacctgggaaggagagaggagtacgacgtgctggacaagcgacgcggacgcgacccggagatgggggggaaaccacggcggaaaaaccctcaggaaggactgtacaacgaactccagaaagacaagatggcggaagcctactcagaaatcgggatgaagggagagcggaggaggggaaagggtcacgacgggctgtaccagggactgagcaccgccactaaggatacctacgatgccttgcatatgcaagcactcccaccccgg

SEQ ID NO: 134 - protein, 492 aa, synthetic construct
  REGION 1..492: note = Description of Artificial Sequence: Synthetic polypeptide
MLLLVTSLLLCELPHPAFLLIPQVQLQQSGPGLVKPSQTLSLTCDISGDSVSSNSAAWNWIRQSPSRGLEWLGRTYYRSKWYNDYAVSVKSRITINPDTSKNQFSLQLNSVTPEDTAVYYCAQEIEPHDAFDIWDQGTMVTVSSGGGGSGGGGSGGGGSVIQMTQSPSSVSASVGDKVTITCRASQDVSGWLAWYQQKPGLAPQLLISGASSLQGGVPSRFSGSGSGTDFTLTISSLQPEDFATYYCQQAKYFPYTFGQGTKLEIKAAATTTPAPRPPTPAPTIASQPLSLRPEACRPAAGGAVHTRGLDFACDIYIWAPLAGTCGVLLLSLVITLYCKRGRKKLLYIFKQPFMRPVQTTQEEDGCSCRFPEEEEGGCELRVKFSRSADAPAYQQGQNQLYNELNLGRREEYDVLDKRRGRDPEMGGKPRRKNPQEGLYNELQKDKMAEAYSEIGMKGERRRGKGHDGLYQGLSTATKDTYDALHMQALPPR

SEQ ID NO: 135 - protein, 6 aa, synthetic construct
  REGION 1..6: note = Description of Artificial Sequence: Synthetic peptide
QDVSGW

SEQ ID NO: 136 - skipped

SEQ ID NO: 137 - protein, 9 aa, synthetic construct
  REGION 1..9: note = Description of Artificial Sequence: Synthetic peptide
QQAKYFPYT

SEQ ID NO: 138 - protein, 10 aa, synthetic construct
  REGION 1..10: note = Description of Artificial Sequence: Synthetic peptide
GDSVSSNSAA

SEQ ID NO: 139 - protein, 9 aa, synthetic construct
  REGION 1..9: note = Description of Artificial Sequence: Synthetic peptide
TYYRSKWYN

SEQ ID NO: 140 - protein, 12 aa, synthetic construct
  REGION 1..12: note = Description of Artificial Sequence: Synthetic peptide
AQEIEPHDAFDI

SEQ ID NO: 141 - DNA, 732 bp, synthetic construct
  misc_feature 1..732: note = Description of Artificial Sequence: Synthetic polynucleotide
  source 1..732: mol_type = other DNA
caagtgcagctgcagcagtccggtcctggactggtcaagcactcccagactctgagcctggcctgcgcgattagcggggactcagtctcgtccaattcggcggcctggaactggatccggcagtcaccatcaaggggcctggaatggctcgggcgcacttactaccggtccaaatggtataacgactacgccgtgtccgtgaagtcccggatcaccattaaccccgacacctcgaagaaccagttctcactccaactgaacagcgtgacccccgaggataccgcggtgtactactgcgcacaagaagtgcagccgcaggacgccctggacatttgggggcagggaacgatggtcacagtgtcgtccggtggaggaggttccggaggcggtggatctggaggcggaggttcggatatccagatgacccagagcccctccttcgtgtccgcatccgtgggcgataaggtcattattacctgtagagcgtcccaggacgtgtccggatggctggcctggtaccagcagaagccaggcttggctcctcaactgctgatctccggcgccagcactcttcagggggaagtgccatcacgcttctccggatccggttccggcaccgacttcaccctgaccatcagcagcctccagcctgaggacttcgccacttactactgccaacaggccaagtacttcccctataccttcggacaaggcactaagctggaaatcaag

SEQ ID NO: 142 - protein, 244 aa, synthetic construct
  REGION 1..244: note = Description of Artificial Sequence: Synthetic polypeptide
QVQLQQSGPGLVKHSQTLSLACAISGDSVSSNSAAWNWIRQSPSRGLEWLGRTYYRSKWYNDYAVSVKSRITINPDTSKNQFSLQLNSVTPEDTAVYYCAQEVQPQDALDIWGQGTMVTVSSGGGGSGGGGSGGGGSDIQMTQSPSFVSASVGDKVIITCRASQDVSGWLAWYQQKPGLAPQLLISGASTLQGEVPSRFSGSGSGTDFTLTISSLQPEDFATYYCQQAKYFPYTFGQGTKLEIK

SEQ ID NO: 143 - DNA, 1476 bp, synthetic construct
  misc_feature 1..1476: note = Description of Artificial Sequence: Synthetic polynucleotide
  source 1..1476: mol_type = other DNA
atgttgctgctcgtgacctcgctccttctgtgcgagctgccccatccggcttttctgctcatccctcaagtgcagctgcagcagtccggtcctggactggtcaagcactcccagactctgagcctggcctgcgcgattagcggggactcagtctcgtccaattcggcggcctggaactggatccggcagtcaccatcaaggggcctggaatggctcgggcgcacttactaccggtccaaatggtataacgactacgccgtgtccgtgaagtcccggatcaccattaaccccgacacctcgaagaaccagttctcactccaactgaacagcgtgacccccgaggataccgcggtgtactactgcgcacaagaagtgcagccgcaggacgccctggacatttgggggcagggaacgatggtcacagtgtcgtccggtggaggaggttccggaggcggtggatctggaggcggaggttcggatatccagatgacccagagcccctccttcgtgtccgcatccgtgggcgataaggtcattattacctgtagagcgtcccaggacgtgtccggatggctggcctggtaccagcagaagccaggcttggctcctcaactgctgatctccggcgccagcactcttcagggggaagtgccatcacgcttctccggatccggttccggcaccgacttcaccctgaccatcagcagcctccagcctgaggacttcgccacttactactgccaacaggccaagtacttcccctataccttcggacaaggcactaagctggaaatcaaggcggccgcaactaccacccctgcccctcggccgccgactccggccccaaccatcgcaagccaacccctctccttgcgccccgaagcttgccgcccggccgcgggtggagccgtgcatacccgggggctggactttgcctgcgatatctacatttgggccccgctggccggcacttgcggcgtgctcctgctgtcgctggtcatcaccctttactgcaagaggggccggaagaagctgctttacatcttcaagcagccgttcatgcggcccgtgcagacgactcaggaagaggacggatgctcgtgcagattccctgaggaggaagaggggggatgcgaactgcgcgtcaagttctcacggtccgccgacgcccccgcatatcaacagggccagaatcagctctacaacgagctgaacctgggaaggagagaggagtacgacgtgctggacaagcgacgcggacgcgacccggagatgggggggaaaccacggcggaaaaaccctcaggaaggactgtacaacgaactccagaaagacaagatggcggaagcctactcagaaatcgggatgaagggagagcggaggaggggaaagggtcacgacgggctgtaccagggactgagcaccgccactaaggatacctacgatgccttgcatatgcaagcactcccaccccgg

SEQ ID NO: 144 - protein, 492 aa, synthetic construct
  REGION 1..492: note = Description of Artificial Sequence: Synthetic polypeptide
MLLLVTSLLLCELPHPAFLLIPQVQLQQSGPGLVKHSQTLSLACAISGDSVSSNSAAWNWIRQSPSRGLEWLGRTYYRSKWYNDYAVSVKSRITINPDTSKNQFSLQLNSVTPEDTAVYYCAQEVQPQDALDIWGQGTMVTVSSGGGGSGGGGSGGGGSDIQMTQSPSFVSASVGDKVIITCRASQDVSGWLAWYQQKPGLAPQLLISGASTLQGEVPSRFSGSGSGTDFTLTISSLQPEDFATYYCQQAKYFPYTFGQGTKLEIKAAATTTPAPRPPTPAPTIASQPLSLRPEACRPAAGGAVHTRGLDFACDIYIWAPLAGTCGVLLLSLVITLYCKRGRKKLLYIFKQPFMRPVQTTQEEDGCSCRFPEEEEGGCELRVKFSRSADAPAYQQGQNQLYNELNLGRREEYDVLDKRRGRDPEMGGKPRRKNPQEGLYNELQKDKMAEAYSEIGMKGERRRGKGHDGLYQGLSTATKDTYDALHMQALPPR

SEQ ID NO: 145 - protein, 6 aa, synthetic construct
  REGION 1..6: note = Description of Artificial Sequence: Synthetic peptide
QDVSGW

SEQ ID NO: 146 - skipped

SEQ ID NO: 147 - protein, 9 aa, synthetic construct
  REGION 1..9: note = Description of Artificial Sequence: Synthetic peptide
QQAKYFPYT

SEQ ID NO: 148 - protein, 10 aa, synthetic construct
  REGION 1..10: note = Description of Artificial Sequence: Synthetic peptide
GDSVSSNSAA

SEQ ID NO: 149 - protein, 9 aa, synthetic construct
  REGION 1..9: note = Description of Artificial Sequence: Synthetic peptide
TYYRSKWYN

SEQ ID NO: 150 - protein, 12 aa, synthetic construct
  REGION 1..12: note = Description of Artificial Sequence: Synthetic peptide
AQEVQPQDALDI

SEQ ID NO: 151 - DNA, 732 bp, synthetic construct
  misc_feature 1..732: note = Description of Artificial Sequence: Synthetic polynucleotide
  source 1..732: mol_type = other DNA
caggtacagctgcagcagtcaggtccaggactggtgaagccctcgcagaccctctcactcacctgtgccatctccggggacagtgtctctagcaacagtgctgcttggaactggatcaggcagtccccatcgagaggccttgagtggctgggaaggacatactacaggtccaagtggtatactgattatgcagtatctgtgaaaaatcgaataaccatcaacccagacacatccaagaatcagttctccctgcagctgaactctgtgactcccgaggacacggctgtgtattactgtgcccaagaggtagaacctcaggatgcttttgatatctggggccaagggacaatggtcaccgtctcttcaggaggtggcgggtctggcggtggaggtagcggtggtggcggatccgacatccagatgacccagtctccatcttccgtgtctgcatctgtaggagacaaagtcaccatcacttgtcgggcgagtcaggatgttagcggctggttagcctggtatcagcagaaaccagggctagcccctcagctcctgatctttggtgcatccactttgcaaggtgaagtcccatcaaggttcagcggcagtggatctgggacagattttactctcaccatcagtagcctgcagcctgaagattttgccacttattattgtcaacaggctaaatatttcccttacacttttggccgggggaccaagctggaaatcaaa

SEQ ID NO: 152 - protein, 244 aa, synthetic construct
  REGION 1..244: note = Description of Artificial Sequence: Synthetic polypeptide
QVQLQQSGPGLVKPSQTLSLTCAISGDSVSSNSAAWNWIRQSPSRGLEWLGRTYYRSKWYTDYAVSVKNRITINPDTSKNQFSLQLNSVTPEDTAVYYCAQEVEPQDAFDIWGQGTMVTVSSGGGGSGGGGSGGGGSDIQMTQSPSSVSASVGDKVTITCRASQDVSGWLAWYQQKPGLAPQLLIFGASTLQGEVPSRFSGSGSGTDFTLTISSLQPEDFATYYCQQAKYFPYTFGRGTKLEIK

SEQ ID NO: 153 - DNA, 1476 bp, synthetic construct
  misc_feature 1..1476: note = Description of Artificial Sequence: Synthetic polynucleotide
  source 1..1476: mol_type = other DNA
atgttgctgctcgtgacctcgctccttctgtgcgagctgccccatccggcttttctgctcatccctcaagtgcagctgcagcagtccggtcctggactggtcaagccgtcccagactctgagcctgacttgcgcaattagcggggactcagtctcgtccaattcggcggcctggaactggatccggcagtcaccatcaaggggcctggaatggctcgggcgcacttactaccggtccaaatggtataccgactacgccgtgtccgtgaagaatcggatcaccattaaccccgacacctcgaagaaccagttctcactccaactgaacagcgtgacccccgaggataccgcggtgtactactgcgcacaagaagtggaaccgcaggacgccttcgacatttggggacagggaacgatggtcacagtgtcgtccggtggaggaggttccggaggcggtggatctggaggcggaggttcggatatccagatgacccagagcccctcctcggtgtccgcatccgtgggcgataaggtcaccattacctgtagagcgtcccaggacgtgtccggatggctggcctggtaccagcagaagccaggcttggctcctcaactgctgatcttcggcgccagcactcttcagggggaagtgccatcacgcttctccggatccggttccggcaccgacttcaccctgaccatcagcagcctccagcctgaggacttcgccacttactactgccaacaggccaagtacttcccctataccttcggaagaggcactaagctggaaatcaaggcggccgcaactaccacccctgcccctcggccgccgactccggccccaaccatcgcaagccaacccctctccttgcgccccgaagcttgccgcccggccgcgggtggagccgtgcatacccgggggctggactttgcctgcgatatctacatttgggccccgctggccggcacttgcggcgtgctcctgctgtcgctggtcatcaccctttactgcaagaggggccggaagaagctgctttacatcttcaagcagccgttcatgcggcccgtgcagacgactcaggaagaggacggatgctcgtgcagattccctgaggaggaagaggggggatgcgaactgcgcgtcaagttctcacggtccgccgacgcccccgcatatcaacagggccagaatcagctctacaacgagctgaacctgggaaggagagaggagtacgacgtgctggacaagcgacgcggacgcgacccggagatgggggggaaaccacggcggaaaaaccctcaggaaggactgtacaacgaactccagaaagacaagatggcggaagcctactcagaaatcgggatgaagggagagcggaggaggggaaagggtcacgacgggctgtaccagggactgagcaccgccactaaggatacctacgatgccttgcatatgcaagcactcccaccccgg

SEQ ID NO: 154 - protein, 492 aa, synthetic construct
  REGION 1..492: note = Description of Artificial Sequence: Synthetic polypeptide
MLLLVTSLLLCELPHPAFLLIPQVQLQQSGPGLVKPSQTLSLTCAISGDSVSSNSAAWNWIRQSPSRGLEWLGRTYYRSKWYTDYAVSVKNRITINPDTSKNQFSLQLNSVTPEDTAVYYCAQEVEPQDAFDIWGQGTMVTVSSGGGGSGGGGSGGGGSDIQMTQSPSSVSASVGDKVTITCRASQDVSGWLAWYQQKPGLAPQLLIFGASTLQGEVPSRFSGSGSGTDFTLTISSLQPEDFATYYCQQAKYFPYTFGRGTKLEIKAAATTTPAPRPPTPAPTIASQPLSLRPEACRPAAGGAVHTRGLDFACDIYIWAPLAGTCGVLLLSLVITLYCKRGRKKLLYIFKQPFMRPVQTTQEEDGCSCRFPEEEEGGCELRVKFSRSADAPAYQQGQNQLYNELNLGRREEYDVLDKRRGRDPEMGGKPRRKNPQEGLYNELQKDKMAEAYSEIGMKGERRRGKGHDGLYQGLSTATKDTYDALHMQALPPR

SEQ ID NO: 155 - protein, 6 aa, synthetic construct
  REGION 1..6: note = Description of Artificial Sequence: Synthetic peptide
QDVSGW

SEQ ID NO: 156 - skipped

SEQ ID NO: 157 - protein, 9 aa, synthetic construct
  REGION 1..9: note = Description of Artificial Sequence: Synthetic peptide
QQAKYFPYT

SEQ ID NO: 158 - protein, 10 aa, synthetic construct
  REGION 1..10: note = Description of Artificial Sequence: Synthetic peptide
GDSVSSNSAA

SEQ ID NO: 159 - protein, 9 aa, synthetic construct
  REGION 1..9: note = Description of Artificial Sequence: Synthetic peptide
TYYRSKWYT

SEQ ID NO: 160 - protein, 12 aa, synthetic construct
  REGION 1..12: note = Description of Artificial Sequence: Synthetic peptide
AQEVEPQDAFDI

SEQ ID NO: 161 - DNA, 732 bp, synthetic construct
  misc_feature 1..732: note = Description of Artificial Sequence: Synthetic polynucleotide
  source 1..732: mol_type = other DNA
caggtacagctgcagcagtcaggtccaggactggtgaagccctcgcagaccctctcactcacctgtgccatctcagggaacagtgtctctagcaacagtgctgcttggaactggatcaggcagtccccatcgagaggccttgagtggctgggaaggacatactacaggtccaagtggtataatgattatgcagtatctgtgaaaagtcgaataaccatcaacccagacacatccaagaaccagttctccctgcagctgaactctgtgactcccgaggacacggctgtgtattactgtgcccaagaggtagaacctcaagatgcttttgatatctggggccaagggacaatggtcaccgtctcttcaggaggtggcgggtctggcggtggaggtagcggtggtggcggatccgacatccagatgacccagtctccatcttccgtgtctgcatctgtaggagacaaagtcaccatcacttgtcgggcgagtcaggatgttagcggctggttagcctggtatcagcagaaaccagggctagcccctcagctcctgatctttggtgcatccactttgcaaggtgaagtcccatcaagattcagcggcggtggatctgggacagattttactctcaccatcagcagcctgcagcctgaagattttgccacttattattgtcaacaggctaaatatttcccttacacttttggccaggggaccaagctggaaatcaaa

SEQ ID NO: 162 - protein, 244 aa, synthetic construct
  REGION 1..244: note = Description of Artificial Sequence: Synthetic polypeptide
QVQLQQSGPGLVKPSQTLSLTCAISGNSVSSNSAAWNWIRQSPSRGLEWLGRTYYRSKWYNDYAVSVKSRITINPDTSKNQFSLQLNSVTPEDTAVYYCAQEVEPQDAFDIWGQGTMVTVSSGGGGSGGGGSGGGGSDIQMTQSPSSVSASVGDKVTITCRASQDVSGWLAWYQQKPGLAPQLLIFGASTLQGEVPSRFSGGGSGTDFTLTISSLQPEDFATYYCQQAKYFPYTFGQGTKLEIK

SEQ ID NO: 163 - DNA, 1476 bp, synthetic construct
  misc_feature 1..1476: note = Description of Artificial Sequence: Synthetic polynucleotide
  source 1..1476: mol_type = other DNA
atgttgctgctcgtgacctcgctccttctgtgcgagctgccccatccggcttttctgctcatccctcaagtgcagctgcagcagtccggtcctggactggtcaagccgtcccagactctgagcctgacttgcgccattagcgggaactcagtctcgtccaattcggcggcctggaactggatccggcagtcaccatcaaggggcctggaatggctcgggcgcacttactaccggtccaaatggtataacgactacgccgtgtccgtgaagtcccggatcaccattaaccccgacacctcgaagaaccagttctcactccaactgaacagcgtgacccccgaggataccgcggtgtactactgcgcacaagaagtggaaccgcaggacgccttcgacatttggggacagggaacgatggtcacagtgtcgtccggtggaggaggttccggaggcggtggatctggaggcggaggttcggatatccagatgacccagagcccctcctcggtgtccgcatccgtgggcgataaggtcaccattacctgtagagcgtcccaggacgtgtccggatggctggcctggtaccagcagaagccaggcttggctcctcaactgctgatctttggcgccagcactcttcagggggaggtgccatcacgcttctccggaggtggttccggcaccgacttcaccctgaccatcagcagcctccagcctgaggacttcgccacttactactgccaacaggccaagtacttcccctataccttcggacaaggcactaagctggaaatcaaggcggccgcaactaccacccctgcccctcggccgccgactccggccccaaccatcgcaagccaacccctctccttgcgccccgaagcttgccgcccggccgcgggtggagccgtgcatacccgggggctggactttgcctgcgatatctacatttgggccccgctggccggcacttgcggcgtgctcctgctgtcgctggtcatcaccctttactgcaagaggggccggaagaagctgctttacatcttcaagcagccgttcatgcggcccgtgcagacgactcaggaagaggacggatgctcgtgcagattccctgaggaggaagaggggggatgcgaactgcgcgtcaagttctcacggtccgccgacgcccccgcatatcaacagggccagaatcagctctacaacgagctgaacctgggaaggagagaggagtacgacgtgctggacaagcgacgcggacgcgacccggagatgggggggaaaccacggcggaaaaaccctcaggaaggactgtacaacgaactccagaaagacaagatggcggaagcctactcagaaatcgggatgaagggagagcggaggaggggaaagggtcacgacgggctgtaccagggactgagcaccgccactaaggatacctacgatgccttgcatatgcaagcactcccaccccgg

SEQ ID NO: 164 - protein, 492 aa, synthetic construct
  REGION 1..492: note = Description of Artificial Sequence: Synthetic polypeptide
MLLLVTSLLLCELPHPAFLLIPQVQLQQSGPGLVKPSQTLSLTCAISGNSVSSNSAAWNWIRQSPSRGLEWLGRTYYRSKWYNDYAVSVKSRITINPDTSKNQFSLQLNSVTPEDTAVYYCAQEVEPQDAFDIWGQGTMVTVSSGGGGSGGGGSGGGGSDIQMTQSPSSVSASVGDKVTITCRASQDVSGWLAWYQQKPGLAPQLLIFGASTLQGEVPSRFSGGGSGTDFTLTISSLQPEDFATYYCQQAKYFPYTFGQGTKLEIKAAATTTPAPRPPTPAPTIASQPLSLRPEACRPAAGGAVHTRGLDFACDIYIWAPLAGTCGVLLLSLVITLYCKRGRKKLLYIFKQPFMRPVQTTQEEDGCSCRFPEEEEGGCELRVKFSRSADAPAYQQGQNQLYNELNLGRREEYDVLDKRRGRDPEMGGKPRRKNPQEGLYNELQKDKMAEAYSEIGMKGERRRGKGHDGLYQGLSTATKDTYDALHMQALPPR

SEQ ID NO: 165 - protein, 6 aa, synthetic construct
  REGION 1..6: note = Description of Artificial Sequence: Synthetic peptide
QDVSGW

SEQ ID NO: 166 - skipped

SEQ ID NO: 167 - protein, 9 aa, synthetic construct
  REGION 1..9: note = Description of Artificial Sequence: Synthetic peptide
QQAKYFPYT

SEQ ID NO: 168 - protein, 10 aa, synthetic construct
  REGION 1..10: note = Description of Artificial Sequence: Synthetic peptide
GNSVSSNSAA

SEQ ID NO: 169 - protein, 9 aa, synthetic construct
  REGION 1..9: note = Description of Artificial Sequence: Synthetic peptide
TYYRSKWYN

SEQ ID NO: 170 - protein, 12 aa, synthetic construct
  REGION 1..12: note = Description of Artificial Sequence: Synthetic peptide
AQEVEPQDAFDI

SEQ ID NO: 171 - DNA, 732 bp, synthetic construct
  misc_feature 1..732: note = Description of Artificial Sequence: Synthetic polynucleotide
  source 1..732: mol_type = other DNA
caggtacagctgcagcagtcaggtccaggactggtgaagccctcgcagaccctctcactcacctgtgccatctccggggacagtgtctctagcaacagtgctgcttggaactggatcaggcagtccccatcgagaggccttgagtggctgggaaggacatactacaggtccaagtggtataatgattatgcagtatctgtgaaaagtcgaataaccatcaacccagacacatccaagaaccagttctccctgcagctgaactctgtgactcccgaggacacggctgtgtattactgtgcccaagaggtagaacctcatgatgctcttgatatctggggccaagggacaatggtcaccgtctcttcaggaggtggcgggtctggcggtggaggtagcggtggtggcggatccgacatccagatgacgcagtctccatcatccgtgtctgcatctgtaggagacaaagtcaccatcacttgtcgggcgagtcaggatgttagcggctggttagcctggtatcaacagaaaccagggctagcccctcagctcctgatctttggtgcatccactttgcaaggtgaagtcccatcaaggttcagcggcagtggatctgggacagattttactctcaccatcagcagcctgcagcctgaagattttgccacttattattgtcaacaggctaaatatttcccttacacttttggccaggggaccaagctggagatcaaa

SEQ ID NO: 172 - protein, 244 aa, synthetic construct; identical to SEQ ID NO: 72
  REGION 1..244: note = Description of Artificial Sequence: Synthetic polypeptide

SEQ ID NO: 173 - DNA, 1476 bp, synthetic construct
  misc_feature 1..1476: note = Description of Artificial Sequence: Synthetic polynucleotide
  source 1..1476: mol_type = other DNA
atgttgctgctcgtgacctcgctccttctgtgcgagctgccccatccggcttttctgctcatccctcaagtgcagctgcagcagtccggtcctggactggtcaagccgtcccagactctgagcctgacttgcgcgattagcggggactcagtctcgtccaattcggcggcctggaactggatccggcagtcaccatcaaggggcctggaatggctcgggcgcacttactaccggtccaaatggtataacgactacgccgtgtccgtgaagtcccggatcaccattaaccccgacacctcgaagaaccagttctcactccaactgaacagcgtgacccccgaggataccgcggtgtactactgcgcacaagaagtggaaccgcacgacgccctggacatttggggtcagggaacgatggtcacagtgtcgtccggtggaggaggttccggaggcggtggatctggaggcggaggttcggatatccagatgacccagagcccctcctcggtgtccgcatccgtgggcgataaggtcaccattacctgtagagcgtcccaggacgtgtccggatggctggcctggtaccagcagaagccaggcttggctcctcaactgctgatcttcggcgccagcacacttcagggggaggtgccatcacgcttctccggatccggttccggcaccgacttcaccctgaccatcagcagcctccagcctgaggacttcgccacttactactgccaacaggccaagtacttcccctataccttcggacaaggcactaagctggaaatcaaggcggccgcaactaccacccctgcccctcggccgccgactccggccccaaccatcgcaagccaacccctctccttgcgccccgaagcttgccgcccggccgcgggtggagccgtgcatacccgggggctggactttgcctgcgatatctacatttgggccccgctggccggcacttgcggcgtgctcctgctgtcgctggtcatcaccctttactgcaagaggggccggaagaagctgctttacatcttcaagcagccgttcatgcggcccgtgcagacgactcaggaagaggacggatgctcgtgcagattccctgaggaggaagaggggggatgcgaactgcgcgtcaagttctcacggtccgccgacgcccccgcatatcaacagggccagaatcagctctacaacgagctgaacctgggaaggagagaggagtacgacgtgctggacaagcgacgcggacgcgacccggagatgggggggaaaccacggcggaaaaaccctcaggaaggactgtacaacgaactccagaaagacaagatggcggaagcctactcagaaatcgggatgaagggagagcggaggaggggaaagggtcacgacgggctgtaccagggactgagcaccgccactaaggatacctacgatgccttgcatatgcaagcactcccaccccgg

SEQ ID NO: 174 - protein, 492 aa, synthetic construct; identical to SEQ ID NO: 74
  REGION 1..492: note = Description of Artificial Sequence: Synthetic polypeptide

SEQ ID NO: 175 - protein, 6 aa, synthetic construct
  REGION 1..6: note = Description of Artificial Sequence: Synthetic peptide
QDVSGW

SEQ ID NO: 176 - skipped

SEQ ID NO: 177 - protein, 9 aa, synthetic construct
  REGION 1..9: note = Description of Artificial Sequence: Synthetic peptide
QQAKYFPYT

SEQ ID NO: 178 - protein, 10 aa, synthetic construct
  REGION 1..10: note = Description of Artificial Sequence: Synthetic peptide
GDSVSSNSAA

SEQ ID NO: 179 - protein, 9 aa, synthetic construct
  REGION 1..9: note = Description of Artificial Sequence: Synthetic peptide
TYYRSKWYN

SEQ ID NO: 180 - protein, 12 aa, synthetic construct
  REGION 1..12: note = Description of Artificial Sequence: Synthetic peptide
AQEVEPHDALDI

SEQ ID NO: 181 - DNA, 66 bp, synthetic construct
  misc_feature 1..66: note = Description of Artificial Sequence: Synthetic oligonucleotide
  source 1..66: mol_type = other DNA
atttgggccccgctggccggcacttgcggcgtgctcctgctgtcgctggtcatcaccctttactgc

SEQ ID NO: 182 - protein, 22 aa, synthetic construct
  REGION 1..22: note = Description of Artificial Sequence: Synthetic peptide
IWAPLAGTCGVLLLSLVITLYC

SEQ ID NO: 183 - DNA, 141 bp, synthetic construct
  misc_feature 1..141: note = Description of Artificial Sequence: Synthetic polynucleotide
  source 1..141: mol_type = other DNA
actaccacccctgcccctcggccgccgactccggccccaaccatcgcaagccaacccctctccttgcgccccgaagcttgccgcccggccgcgggtggagccgtgcatacccgggggctggactttgcctgcgatatctac

SEQ ID NO: 184 - protein, 47 aa, synthetic construct
  REGION 1..47: note = Description of Artificial Sequence: Synthetic polypeptide
TTTPAPRPPTPAPTIASQPLSLRPEACRPAAGGAVHTRGLDFACDIY

SEQ ID NO: 185 - protein, 69 aa, synthetic construct
  REGION 1..69: note = Description of Artificial Sequence: Synthetic polypeptide
TTTPAPRPPTPAPTIASQPLSLRPEACRPAAGGAVHTRGLDFACDIYIWAPLAGTCGVLLLSLVITLYC

SEQ ID NO: 186 - DNA, 126 bp, synthetic construct
  misc_feature 1..126: note = Description of Artificial Sequence: Synthetic polynucleotide
  source 1..126: mol_type = other DNA
aagaggggccggaagaagctgctttacatcttcaagcagccgttcatgcggcccgtgcagacgactcaggaagaggacggatgctcgtgcagattccctgaggaggaagaggggggatgcgaactg

SEQ ID NO: 187 - protein, 42 aa, synthetic construct
  REGION 1..42: note = Description of Artificial Sequence: Synthetic polypeptide
KRGRKKLLYIFKQPFMRPVQTTQEEDGCSCRFPEEEEGGCEL

SEQ ID NO: 188 - DNA, 336 bp, synthetic construct
  misc_feature 1..336: note = Description of Artificial Sequence: Synthetic polynucleotide
  source 1..336: mol_type = other DNA
cgcgtcaagttctcacggtccgccgacgcccccgcatatcaacagggccagaatcagctctacaacgagctgaacctgggaaggagagaggagtacgacgtgctggacaagcgacgcggacgcgacccggagatgggggggaaaccacggcggaaaaaccctcaggaaggactgtacaacgaactccagaaagacaagatggcggaagcctactcagaaatcgggatgaagggagagcggaggaggggaaagggtcacgacgggctgtaccagggactgagcaccgccactaaggatacctacgatgccttgcatatgcaagcactcccaccccgg

SEQ ID NO: 189 - protein, 112 aa, synthetic construct
  REGION 1..112: note = Description of Artificial Sequence: Synthetic polypeptide
RVKFSRSADAPAYQQGQNQLYNELNLGRREEYDVLDKRRGRDPEMGGKPRRKNPQEGLYNELQKDKMAEAYSEIGMKGERRRGKGHDGLYQGLSTATKDTYDALHMQALPPR

SEQ ID NO: 190 - DNA, 66 bp, synthetic construct
  misc_feature 1..66: note = Description of Artificial Sequence: Synthetic oligonucleotide
  source 1..66: mol_type = other DNA
atgctgctgctggtgaccagcctgctgctgtgcgaactgccgcatccggcgtttctgctgattccg

SEQ ID NO: 191 - protein, 22 aa, synthetic construct
  REGION 1..22: note = Description of Artificial Sequence: Synthetic peptide
MLLLVTSLLLCELPHPAFLLIP

SEQ ID NO: 192 - DNA, 726 bp, synthetic construct
  misc_feature 1..726: note = Description of Artificial Sequence: Synthetic polynucleotide
  source 1..726: mol_type = other DNA
gacattcagatgactcagaccacctcttccttgtccgcgtcactgggagacagagtgaccatctcgtgtcgcgcaagccaggatatctccaagtacctgaactggtaccaacagaagcccgacgggactgtgaagctgctgatctaccacacctcacgcctgcacagcggagtgccaagcagattctccggctccggctcgggaaccgattactcgcttaccattagcaacctcgagcaggaggacatcgctacctacttctgccagcaaggaaataccctgccctacaccttcggcggaggaaccaaattggaaatcaccggcggaggaggctccgggggaggaggttccgggggcgggggttccgaagtgaagctccaggagtccggccccggcctggtggcgccgtcgcaatcactctctgtgacctgtaccgtgtcgggagtgtccctgcctgattacggcgtgagctggattcggcagccgccgcggaagggcctggaatggctgggtgtcatctggggatccgagactacctactacaactcggccctgaagtcccgcctgactatcatcaaagacaactcgaagtcccaggtctttctgaagatgaactccctgcaaactgacgacaccgccatctattactgtgctaagcactactactacggtggaagctatgctatggactactgggggcaaggcacttcggtgactgtgtcaagc

SEQ ID NO: 193 - protein, 242 aa, synthetic construct
  REGION 1..242: note = Description of Artificial Sequence: Synthetic polypeptide
DIQMTQTTSSLSASLGDRVTISCRASQDISKYLNWYQQKPDGTVKLLIYHTSRLHSGVPSRFSGSGSGTDYSLTISNLEQEDIATYFCQQGNTLPYTFGGGTKLEITGGGGSGGGGSGGGGSEVKLQESGPGLVAPSQSLSVTCTVSGVSLPDYGVSWIRQPPRKGLEWLGVIWGSETTYYNSALKSRLTIIKDNSKSQVFLKMNSLQTDDTAIYYCAKHYYYGGSYAMDYWGQGTSVTVSS

SEQ ID NO: 194 - DNA, 1470 bp, synthetic construct
  misc_feature 1..1470: note = Description of Artificial Sequence: Synthetic polynucleotide
  source 1..1470: mol_type = other DNA
atgcttctcctggtcacctccctgctcctctgcgaactgcctcaccctgccttccttctgattcctgacattcagatgactcagaccacctcttccttgtccgcgtcactgggagacagagtgaccatctcgtgtcgcgcaagccaggatatctccaagtacctgaactggtaccaacagaagcccgacgggactgtgaagctgctgatctaccacacctcacgcctgcacagcggagtgccaagcagattctccggctccggctcgggaaccgattactcgcttaccattagcaacctcgagcaggaggacatcgctacctacttctgccagcaaggaaataccctgccctacaccttcggcggaggaaccaaattggaaatcaccggcggaggaggctccgggggaggaggttccgggggcgggggttccgaagtgaagctccaggagtccggccccggcctggtggcgccgtcgcaatcactctctgtgacctgtaccgtgtcgggagtgtccctgcctgattacggcgtgagctggattcggcagccgccgcggaagggcctggaatggctgggtgtcatctggggatccgagactacctactacaactcggccctgaagtcccgcctgactatcatcaaagacaactcgaagtcccaggtctttctgaagatgaactccctgcaaactgacgacaccgccatctattactgtgctaagcactactactacggtggaagctatgctatggactactgggggcaaggcacttcggtgactgtgtcaagcgcggccgcaactaccacccctgcccctcggccgccgactccggccccaaccatcgcaagccaacccctctccttgcgccccgaagcttgccgcccggccgcgggtggagccgtgcatacccgggggctggactttgcctgcgatatctacatttgggccccgctggccggcacttgcggcgtgctcctgctgtcgctggtcatcaccctttactgcaagaggggccggaagaagctgctttacatcttcaagcagccgttcatgcggcccgtgcagacgactcaggaagaggacggatgctcgtgcagattccctgaggaggaagaggggggatgcgaactgcgcgtcaagttctcacggtccgccgacgcccccgcatatcaacagggccagaatcagctctacaacgagctgaacctgggaaggagagaggagtacgacgtgctggacaagcgacgcggacgcgacccggagatgggggggaaaccacggcggaaaaaccctcaggaaggactgtacaacgaactccagaaagacaagatggcggaagcctactcagaaatcgggatgaagggagagcggaggaggggaaagggtcacgacgggctgtaccagggactgagcaccgccactaaggatacctacgatgccttgcatatgcaagcactcccaccccgg

SEQ ID NO: 195 - protein, 490 aa, synthetic construct
  REGION 1..490: note = Description of Artificial Sequence: Synthetic polypeptide
MLLLVTSLLLCELPHPAFLLIPDIQMTQTTSSLSASLGDRVTISCRASQDISKYLNWYQQKPDGTVKLLIYHTSRLHSGVPSRFSGSGSGTDYSLTISNLEQEDIATYFCQQGNTLPYTFGGGTKLEITGGGGSGGGGSGGGGSEVKLQESGPGLVAPSQSLSVTCTVSGVSLPDYGVSWIRQPPRKGLEWLGVIWGSETTYYNSALKSRLTIIKDNSKSQVFLKMNSLQTDDTAIYYCAKHYYYGGSYAMDYWGQGTSVTVSSAAATTTPAPRPPTPAPTIASQPLSLRPEACRPAAGGAVHTRGLDFACDIYIWAPLAGTCGVLLLSLVITLYCKRGRKKLLYIFKQPFMRPVQTTQEEDGCSCRFPEEEEGGCELRVKFSRSADAPAYQQGQNQLYNELNLGRREEYDVLDKRRGRDPEMGGKPRRKNPQEGLYNELQKDKMAEAYSEIGMKGERRRGKGHDGLYQGLSTATKDTYDALHMQALPPR

SEQ ID NO: 196 - DNA, 1482 bp, synthetic construct
  misc_feature 1..1482: note = Description of Artificial Sequence: Synthetic polynucleotide
  source 1..1482: mol_type = other DNA
atgcttcttttggtgacttcccttttgctgtgcgagttgccacaccccgccttcctgcttattccccaggtacagctccagcagagtggcccagggctcgtgaagccaagccagacgctgtccctgacttgtgcaatttcaggggattcagtttcatcaaatagcgcggcgtggaattggattcgacaatctccttcccgagggttggaatggcttggacgaacatattacagatccaaatggtataacgactatgcggtatcagtaaagtcaagaataaccattaaccccgacacaagcaagaaccaattctctttgcagcttaactctgtcacgccagaagacacggcagtctattattgcgctcgcgaggtaacgggtgacctggaagacgcttttgacatttgggggcagggtacgatggtgacagtcagttcagggggcggtgggagtgggggagggggtagcggggggggagggtcagacattcagatgacccagtccccttcatccttgtctgcctccgtcggtgacagggtgacaataacatgcagagcaagccaaacaatctggagctatctcaactggtaccagcagcgaccaggaaaagcgccaaacctgctgatttacgctgcttcctccctccaatcaggcgtgcctagtagatttagcggtaggggctccggcaccgattttacgctcactataagctctcttcaagcagaagattttgcgacttattactgccagcagtcctatagtatacctcagactttcggacagggtaccaagttggagattaaggcggccgcaactaccacccctgcccctcggccgccgactccggccccaaccatcgcaagccaacccctctccttgcgccccgaagcttgccgcccggccgcgggtggagccgtgcatacccgggggctggactttgcctgcgatatctacatttgggccccgctggccggcacttgcggcgtgctcctgctgtcgctggtcatcaccctttactgcaagaggggccggaagaagctgctttacatcttcaagcagccgttcatgcggcccgtgcagacgactcaggaagaggacggatgctcgtgcagattccctgaggaggaagaggggggatgcgaactgcgcgtcaagttctcacggtccgccgacgcccccgcatatcaacagggccagaatcagctctacaacgagctgaacctgggaaggagagaggagtacgacgtgctggacaagcgacgcggacgcgacccggagatgggggggaaaccacggcggaaaaaccctcaggaaggactgtacaacgaactccagaaagacaagatggcggaagcctactcagaaatcgggatgaagggagagcggaggaggggaaagggtcacgacgggctgtaccagggactgagcaccgccactaaggatacctacgatgccttgcatatgcaagcactcccaccccgg

SEQ ID NO: 197 - protein, 494 aa, synthetic construct
  REGION 1..494: note = Description of Artificial Sequence: Synthetic polypeptide
MLLLVTSLLLCELPHPAFLLIPQVQLQQSGPGLVKPSQTLSLTCAISGDSVSSNSAAWNWIRQSPSRGLEWLGRTYYRSKWYNDYAVSVKSRITINPDTSKNQFSLQLNSVTPEDTAVYYCAREVTGDLEDAFDIWGQGTMVTVSSGGGGSGGGGSGGGGSDIQMTQSPSSLSASVGDRVTITCRASQTIWSYLNWYQQRPGKAPNLLIYAASSLQSGVPSRFSGRGSGTDFTLTISSLQAEDFATYYCQQSYSIPQTFGQGTKLEIKAAATTTPAPRPPTPAPTIASQPLSLRPEACRPAAGGAVHTRGLDFACDIYIWAPLAGTCGVLLLSLVITLYCKRGRKKLLYIFKQPFMRPVQTTQEEDGCSCRFPEEEEGGCELRVKFSRSADAPAYQQGQNQLYNELNLGRREEYDVLDKRRGRDPEMGGKPRRKNPQEGLYNELQKDKMAEAYSEIGMKGERRRGKGHDGLYQGLSTATKDTYDALHMQALPPR

SEQ ID NO: 198 - DNA, 732 bp, synthetic construct
  misc_feature 1..732: note = Description of Artificial Sequence: Synthetic polynucleotide
  source 1..732: mol_type = other DNA
gaggtccagctggtacagtctgggggaggcttggtacagcctggggggtccctgagactctcctgtgcagcctctggattcacctttgatgattatgccatgcactgggtccggcaagctccagggaagggcctggagtgggtctcaggtattagttggaatagtggtagcataggctatgcggactctgtgaagggccgattcaccatctccagagacaacgccaagaactccctgtatctgcaaatgaacagtctgagagctgaggacacggccttgtattactgtgcaaaagatttatcgtcagtggctggaccctttaactactggggccagggcaccctggtcaccgtctcctcaggaggtggcgggtctggtggaggcggtagcggcggtggcggatcctcttctgagctgactcaggaccctgctgtgtctgtggccttgggacagacagtcaggatcacatgccaaggagacagcctcagaagctattatgcaagctggtaccagcagaagccaggacaggcccctgtacttgtcatctatggtaaaaacaaccggccctcagggatcccagaccgattctctggctccagctcaggaaacacagcttccttgaccatcactggggctcaggcggaggatgaggctgactattactgtaactcccgggacagcagtggtaaccatctggtattcggcggaggcacccagctgaccgtcctcggt

SEQ ID NO: 199 - protein, 244 aa, synthetic construct
  REGION 1..244: note = Description of Artificial Sequence: Synthetic polypeptide
EVQLVQSGGGLVQPGGSLRLSCAASGFTFDDYAMHWVRQAPGKGLEWVSGISWNSGSIGYADSVKGRFTISRDNAKNSLYLQMNSLRAEDTALYYCAKDLSSVAGPFNYWGQGTLVTVSSGGGGSGGGGSGGGGSSSELTQDPAVSVALGQTVRITCQGDSLRSYYASWYQQKPGQAPVLVIYGKNNRPSGIPDRFSGSSSGNTASLTITGAQAEDEADYYCNSRDSSGNHLVFGGGTQLTVLG

SEQ ID NO: 200 - DNA, 1476 bp, synthetic construct
  misc_feature 1..1476: note = Description of Artificial Sequence: Synthetic polynucleotide
  source 1..1476: mol_type = other DNA
atgctgctgctggtgaccagcctgctgctgtgcgaactgccgcatccggcgtttctgctgattccggaggtccagctggtacagtctgggggaggcttggtacagcctggggggtccctgagactctcctgtgcagcctctggattcacctttgatgattatgccatgcactgggtccggcaagctccagggaagggcctggagtgggtctcaggtattagttggaatagtggtagcataggctatgcggactctgtgaagggccgattcaccatctccagagacaacgccaagaactccctgtatctgcaaatgaacagtctgagagctgaggacacggccttgtattactgtgcaaaagatttatcgtcagtggctggaccctttaactactggggccagggcaccctggtcaccgtctcctcaggaggtggcgggtctggtggaggcggtagcggcggtggcggatcctcttctgagctgactcaggaccctgctgtgtctgtggccttgggacagacagtcaggatcacatgccaaggagacagcctcagaagctattatgcaagctggtaccagcagaagccaggacaggcccctgtacttgtcatctatggtaaaaacaaccggccctcagggatcccagaccgattctctggctccagctcaggaaacacagcttccttgaccatcactggggctcaggcggaggatgaggctgactattactgtaactcccgggacagcagtggtaaccatctggtattcggcggaggcacccagctgaccgtcctcggtgcggccgcaactaccacccctgcccctcggccgccgactccggccccaaccatcgcaagccaacccctctccttgcgccccgaagcttgccgcccggccgcgggtggagccgtgcatacccgggggctggactttgcctgcgatatctacatttgggccccgctggccggcacttgcggcgtgctcctgctgtcgctggtcatcaccctttactgcaagaggggccggaagaagctgctttacatcttcaagcagccgttcatgcggcccgtgcagacgactcaggaagaggacggatgctcgtgcagattccctgaggaggaagaggggggatgcgaactgcgcgtcaagttctcacggtccgccgacgcccccgcatatcaacagggccagaatcagctctacaacgagctgaacctgggaaggagagaggagtacgacgtgctggacaagcgacgcggacgcgacccggagatgggggggaaaccacggcggaaaaaccctcaggaaggactgtacaacgaactccagaaagacaagatggcggaagcctactcagaaatcgggatgaagggagagcggaggaggggaaagggtcacgacgggctgtaccagggactgagcaccgccactaaggatacctacgatgccttgcatatgcaagcactcccaccccgg

SEQ ID NO: 201 - protein, 492 aa, synthetic construct
  REGION 1..492: note = Description of Artificial Sequence: Synthetic polypeptide
MLLLVTSLLLCELPHPAFLLIPEVQLVQSGGGLVQPGGSLRLSCAASGFTFDDYAMHWVRQAPGKGLEWVSGISWNSGSIGYADSVKGRFTISRDNAKNSLYLQMNSLRAEDTALYYCAKDLSSVAGPFNYWGQGTLVTVSSGGGGSGGGGSGGGGSSSELTQDPAVSVALGQTVRITCQGDSLRSYYASWYQQKPGQAPVLVIYGKNNRPSGIPDRFSGSSSGNTASLTITGAQAEDEADYYCNSRDSSGNHLVFGGGTQLTVLGAAATTTPAPRPPTPAPTIASQPLSLRPEACRPAAGGAVHTRGLDFACDIYIWAPLAGTCGVLLLSLVITLYCKRGRKKLLYIFKQPFMRPVQTTQEEDGCSCRFPEEEEGGCELRVKFSRSADAPAYQQGQNQLYNELNLGRREEYDVLDKRRGRDPEMGGKPRRKNPQEGLYNELQKDKMAEAYSEIGMKGERRRGKGHDGLYQGLSTATKDTYDALHMQALPPR

SEQ ID NO: 202 - DNA, 339 bp, synthetic construct
  misc_feature 1..339: note = Description of Artificial Sequence: Synthetic polynucleotide
  source 1..339: mol_type = other DNA
gaggtgcagctggtggagtctgggggaggcttggtacagcctggagggtccctgagactctcctgtgcagcctctggattcaccttcagtagctatggcatgagctgggtccgccaggctccaagacaagggcttgagtgggtggccaacataaagcaagatggaagtgagaaatactatgcggactcagtgaagggccgattcaccatctccagagacaattccaagaacacgctgtatctgcaaatgaacagcctgagagccgaggacacagccacgtattactgtgcgaaagaaaatgtggactggggccagggcaccctggtcaccgtctcctca

SEQ ID NO: 203 - protein, 113 aa, synthetic construct
  REGION 1..113: note = Description of Artificial Sequence: Synthetic polypeptide
EVQLVESGGGLVQPGGSLRLSCAASGFTFSSYGMSWVRQAPRQGLEWVANIKQDGSEKYYADSVKGRFTISRDNSKNTLYLQMNSLRAEDTATYYCAKENVDWGQGTLVTVSS

SEQ ID NO: 204 - DNA, 1083 bp, synthetic construct
  misc_feature 1..1083: note = Description of Artificial Sequence: Synthetic polynucleotide
  source 1..1083: mol_type = other DNA
atgctgctgctggtgaccagcctgctgctgtgcgaactgccgcatccggcgtttctgctgattccggaggtgcagctggtggagtctgggggaggcttggtacagcctggagggtccctgagactctcctgtgcagcctctggattcaccttcagtagctatggcatgagctgggtccgccaggctccaagacaagggcttgagtgggtggccaacataaagcaagatggaagtgagaaatactatgcggactcagtgaagggccgattcaccatctccagagacaattccaagaacacgctgtatctgcaaatgaacagcctgagagccgaggacacagccacgtattactgtgcgaaagaaaatgtggactggggccagggcaccctggtcaccgtctcctcagcggccgcaactaccacccctgcccctcggccgccgactccggccccaaccatcgcaagccaacccctctccttgcgccccgaagcttgccgcccggccgcgggtggagccgtgcatacccgggggctggactttgcctgcgatatctacatttgggccccgctggccggcacttgcggcgtgctcctgctgtcgctggtcatcaccctttactgcaagaggggccggaagaagctgctttacatcttcaagcagccgttcatgcggcccgtgcagacgactcaggaagaggacggatgctcgtgcagattccctgaggaggaagaggggggatgcgaactgcgcgtcaagttctcacggtccgccgacgcccccgcatatcaacagggccagaatcagctctacaacgagctgaacctgggaaggagagaggagtacgacgtgctggacaagcgacgcggacgcgacccggagatgggggggaaaccacggcggaaaaaccctcaggaaggactgtacaacgaactccagaaagacaagatggcggaagcctactcagaaatcgggatgaagggagagcggaggaggggaaagggtcacgacgggctgtaccagggactgagcaccgccactaaggatacctacgatgccttgcatatgcaagcactcccaccccgg

SEQ ID NO: 205 - protein, 361 aa, synthetic construct
  REGION 1..361: note = Description of Artificial Sequence: Synthetic polypeptide
MLLLVTSLLLCELPHPAFLLIPEVQLVESGGGLVQPGGSLRLSCAASGFTFSSYGMSWVRQAPRQGLEWVANIKQDGSEKYYADSVKGRFTISRDNSKNTLYLQMNSLRAEDTATYYCAKENVDWGQGTLVTVSSAAATTTPAPRPPTPAPTIASQPLSLRPEACRPAAGGAVHTRGLDFACDIYIWAPLAGTCGVLLLSLVITLYCKRGRKKLLYIFKQPFMRPVQTTQEEDGCSCRFPEEEEGGCELRVKFSRSADAPAYQQGQNQLYNELNLGRREEYDVLDKRRGRDPEMGGKPRRKNPQEGLYNELQKDKMAEAYSEIGMKGERRRGKGHDGLYQGLSTATKDTYDALHMQALPPR

SEQ ID NO: 206 - protein, 4 aa, synthetic construct
  REGION 1..4: note = Description of Artificial Sequence: Synthetic peptide
GFLG